European Patent Specification EP 3 672 605 B1, published October 23, 2024. Title: PRE-NATAL TRANSPLANTATION OF FACTOR VIII-EXPRESSING CELLS FOR TREATMENT OF HEMOPHILIA. Applicant: Wake Forest University Health Sciences Emory University Children's Healthcare of Atlanta, Inc. The sequence listing filed with the application follows.

SEQUENCE LISTING (33 sequences)

SEQ ID NO: 1 - DNA, 146 bp, Artificial Sequence
  synthetic HNF1-shortABP-SynO-TSS
gttaatcattaagtcgttaatttttgtggcccttgcgatgtttgctctggttaataatctcaggacaaacagaggttaataattttccagatctctctgagcaatagtataaaaggccagcagcagcctgaccacatctcatcctc

SEQ ID NO: 2 - DNA, 159 bp, Artificial Sequence
  synthetic ABPshort-HP1-AFP-TSS
gttaatttttgtggcccttgcgatgtttgctctggttaataatctcaggacaaacatacattttcagtcatatgtttgctcactgaaggttactagttaacaggcatcccttaaacaggatataaaaggccagcagcagcctgaccacatctcatcctc

SEQ ID NO: 3 - DNA, 152 bp, Artificial Sequence
  HNF1-ABP-SynO
gttaatcattaagtcgttaatttttaaaaagcagtcaaaagtccaagtggcccttgcgagcatttactctctctgtttgctctggttaataatctcaggagcacaaacagaggttaataattttccagatctctctgagcaatagtataaaa

SEQ ID NO: 4 - DNA, 150 bp, Artificial Sequence
  synthetic SP1-ABP-SynO
tgggcggagtgtcgttaatttttaaaaagcagtcaaaagtccaagtggcccttgcgagcatttactctctctgtttgctctggttaataatctcaggagcacaaacagaggttaataattttccagatctctctgagcaatagtataaaa

SEQ ID NO: 5 - DNA, 137 bp, Artificial Sequence
  synthetic ABP-SynO
gttaatttttaaaaagcagtcaaaagtccaagtggcccttgcgagcatttactctctctgtttgctctggttaataatctcaggagcacaaacagaggttaataattttccagatctctctgagcaatagtataaaa

SEQ ID NO: 6 - DNA, 172 bp, Artificial Sequence
  synthetic ABP-HP1-AFP
gttaatttttaaaaagcagtcaaaagtccaagtggcccttgcgagcatttactctctctgtttgctctggttaataatctcaggagcacaaacagaggttaataattttcagtcatatgtttgctcactgaaggttactagttaacaggcatcccttaaacaggatataaaa

SEQ ID NO: 7 - DNA, 4377 bp, Artificial Sequence
  synthetic hcoAn53
atgcagattgagctgtccacttgctttttcctgtgcctgctgcagttttcattttccgccactagaagatactacctgggggctgtcgaactgtcctgggattacatgcagtccgacctgctgtctgagctgcatgtggacacccgatttccacctcgcgtcccacgaagcttcccctttaatacatccgtgatgtacaagaaaactgtgttcgtcgagttcaccgatcacctgttcaacatcgcaaagccccggccaccctggatgggactgctgggccctaccatcagagccgaggtgtacgacaccgtggtcattacactgaaaaacatggcaagtcaccccgtgtcactgcatgccgtgggagtctcctactggaaggcatctgaaggcgccgagtatgacgatcagactagtcagagagaaaaagaggacgataaggtgtttcccggagaatctcatacctatgtgtggcaggtcctgaaggagaatggccctatggccagcgaccctccatgcctgacctactcctatctgtctcacgtggacctggtcaaagatctgaactccgggctgatcggagccctgctggtgtgtcgggaaggatctctggctaaggagagaacccagacactgcatcagttcgtgctgctgttcgctgtctttgacgaaggcaaaagttggcactcagagacaaaggattccctgactcaggcaatggactctgccagtgctagggcatggccaaaaatgcacaccgtgaacggctacgtcaatagaagcctgccaggactgatcggatgccacaggaagtccgtgtattggcatgtcatcggcatggggaccacaccagaagtccactctattttcctggagggacatacatttctggtgcggaatcacagacaggctagcctggagatctcccccattaccttcctgacagcacagactctgctgatggatctgggccagttcctgctgttttgccacatcagctcccaccagcatgatgggatggaggcctacgtgaaagtcgacagctgtccagaggaaccccagctgaggatgaagaacaatgaggaagaggaagactacgacgatgacctgtatgacagcgagatggatgtggtccgattcgatgacgataactcacccccttttatccagattagaagcgtcgccaagaaacaccctaagacttgggtgcattacatcgccgctgaggaagaggactgggattatgctccttccgtgctgaccccagacgatcgcagctacaaatcccagtatctgaacaatggccctcagaggattgggcgcaagtacaagaaagtgaggttcatggcttataccgatgaaaccttcaagactcgcgaagcaatccagtacgagtccggaattctgggcccactgctgtatggggaagtgggagacaccctgctgatcattttcaagaaccaggcctctaggccctacaatatctatcctcatggcattacagatgtgtctcccctgcacagtggacgcctgcctaagggcgtgaaacacctgaaggacctgcctatcctgccaggggaaatttttaagtacaaatggactgtgaccgtcgaggatggaccaactaagagcgaccccaggtgcctgacccgctactattctagtttcatcaatctggaaagagatctggcaagcggactgatcggaccactgctgatttgttacaaagagtccgtggatcagcgaggcaaccagatgatgtctgacaagcggaatgtgatcctgttctcagtctttgacgaaaaccgcagctggtatctgaccgagaacatgcagcgattcctgccaaatgcagcaggagtgcagccacaggatcctgagtttcaggctagtaacatcatgcattcaattaatggctacgtgttcgactcactgcagctgagcgtgtgtctgcacgaggtcgcttactggtatatcctgagcgtcggagcacagacagatttcctgtccgtgttcttttctggctacacttttaagcataaaatggtgtatgaggacacactgactctgttccctttttccggcgaaaccgtctttatgtctatggagaatccagggctgtgggtgctgggatgccacaactccgatttccggaatagaggaatgactgccctgctgaaagtgtcaagctgtgaccggaacaccggcgactactatgaagatacatacgaggacatcccaacttatctgctgtctgaaaacaatgtgattgagcccagaagcttcagccagaatccacccgtgctgaagcgacaccagcgggaaatcaccctgactaccctgcagtcagagcaggaagagattgattacgacgataccatcagcattgaaacaaaaagggaggacttcgatatctatggggaagacgagaaccagggacctcgctccttccagaagaggacacgccattactttattgctgcagtggagaggctgtgggattatgggatgtcccgctctccccacgtcctgcgaaatcgggcccagagtggatcagtgcctcagttcaagaaagtggtcttccaggagtttactgacgggagctttacccagcctctgtaccggggagaactgaacgagcacctgggactgctgggcccatatatcagagcagaagtggaggataacattatggtcaccttcaagaatcaggccagtcggccctactcattttattcctctctgatcagctacgaagaggaccagcgccagggcgcagaaccacgaaaaaacttcgtgaagcccaatgagaccaaaacatacttttggaaggtgcagcaccatatggctcctacaaaagacgaattcgattgcaaggcctgggcttattttagtgacgtggatctggagaaggacatgcactcagggctgatcggacctctgctgatttgtcatactaacaccctgaatccagcacacggacgacaggtgacagtccaggaattcgctctgttctttacaatcttcgatgagactaagagctggtacttcactgaaaacatggagagaaattgcagggccccttgtaatatccagatggaagacccaacattcaaggagaactacagatttcatgctattaatggctatgtgatggatactctgccagggctggtcatggcacaggaccagagaatcaggtggtacctgctgtctatggggagtaacgagaatatccacagcattcatttctccggacacgtgtttactgtcaggaagaaagaagagtataaaatggccgtgtacaacctgtatccaggcgtgttcgaaaccgtcgagatgctgccaagcaaggcaggaatctggcgagtggaatgcctgattggcgagcacctgcatgctgggatgagtaccctgtttctggtgtactcaaaacagtgtcagacacctctgggaatggcatctggccatatccgggatttccagattaccgcaagtggacagtacggacagtgggctccaaagctggcaagactgcactatagcggctccatcaacgcctggtctacaaaagagccctttagttggattaaggtggacctgctggcccctatgatcattcatggcatcaaaactcagggggctaggcagaagttcagttcactgtacatcagccagtttatcatcatgtactccctggatgggaagaaatggcagacctaccgcgggaatagcacaggaactctgatggtgttctttggaaacgtcgacagctccggcatcaagcacaacattttcaatcctccaatcattgcccgctacatccgactgcaccccacccattattcaattcgaagcacactgcggatggaactgatgggctgcgatctgaactcttgtagtatgcctctggggatggagtctaaggccatcagtgacgctcagattaccgcatctagttacttcaccaatatgtttgccacatggtcaccaagccaggctaggctgcacctgcagggaagaacaaacgcctggaggcctcaggtgaacaatccaaaggagtggctgcaggtggatttccagaaaactatgaaggtcaccggaatcacaactcagggcgtgaaatcactgctgaccagcatgtatgtgaaggagtttctgatttcaagctcccaggacggccaccattggacactgttcctgcagaacgggaaggtgaaagtcttccagggaaatcaggattcttttacaccagtggtcaacagtctggacccccctctgctgactcggtacctgagaatccacccccagagctgggtccatcagattgcactgcgactggaagtgctgggatgcgaggcacagcagctgtattga

SEQ ID NO: 8 - DNA, 4359 bp, Artificial Sequence
  synthetic lcoAn53
atgcagattgagctgagcacctgcttcttcctgtgcctgctgcagttctcattctctgccaccaggagatactacctgggcgccgtggagctgagctgggactacatgcagtctgacctgctgtctgagctgcatgtggacaccaggttcccccccagagtgccccgaagcttccccttcaacaccagcgtgatgtacaagaagaccgtgttcgtggagttcactgaccacctgttcaacatcgccaagcccaggcccccctggatgggcctgctgggccccaccatcagagccgaggtgtacgacaccgtggtcatcaccctgaagaacatggccagccaccccgtctccctgcacgccgtgggggtgagctactggaaggcctctgagggcgccgagtacgacgaccagaccagccagagggagaaggaggacgacaaggtgttccctggggaaagccacacctacgtgtggcaggtcctgaaggagaacggccccatggcctctgaccccccatgcctgacctacagctacctgagccacgtggacctggtgaaggacctgaactctggcctgattggggccctgctggtgtgcagggagggcagcctggccaaggagagaacccagaccctgcaccagttcgtgctgctgttcgccgtgttcgacgagggcaagagctggcactctgaaaccaaggatagcctgactcaggccatggactctgcctctgccagggcctggcccaagatgcacaccgtcaacggctacgtcaacaggagcctgcctggcctgattggctgccacaggaagagcgtgtactggcatgtgatcggcatgggcaccacccctgaggtgcacagcatcttcctggagggccacaccttcctggtcaggaaccacaggcaggccagcctggagatcagccccatcaccttcctgaccgcccagaccctgctgatggacctgggccagttcctgctgttctgccacatctccagccaccagcacgacggcatggaggcctacgtgaaagtggacagctgccctgaggagccccagctgaggatgaagaacaacgaggaggaggaggactatgatgacgacctgtatgacagcgagatggacgtggtcaggttcgacgacgacaacagcccccctttcatccagatcaggagcgtggccaagaagcaccccaagacctgggtgcactacatcgctgctgaggaggaggactgggactatgccccctccgtgctgacccctgatgacaggagctacaagagccagtacctgaacaatggcccccagaggattggcaggaagtacaagaaagtcaggttcatggcctacactgatgaaaccttcaagaccagggaggccatccagtacgagtctggcatcctgggccccctgctgtacggggaggtgggggacaccctgctgatcatcttcaagaaccaggccagcaggccctacaacatctacccccatggcatcaccgacgtgagccccctgcacagcggaaggctgcctaagggggtgaagcacctgaaagacctgcccatcctgcctggggagatcttcaagtacaagtggactgtgactgtggaggacggccccaccaagagcgaccccaggtgcctgaccagatactacagcagcttcatcaacctggagagggacctggcctctggcctgattggccccctgctgatctgctacaaggagtctgtggaccagaggggcaaccagatgatgagcgacaagaggaacgtgatcctgttctctgtcttcgacgagaacaggagctggtacctgaccgagaacatgcagaggttcctgcccaacgcagctggggtgcagccacaggaccccgagttccaggccagcaacatcatgcacagcatcaatggctacgtgttcgacagcctgcagctgagcgtgtgcctgcacgaggtggcctactggtacatcctgagcgtcggcgcccagaccgacttcctgagcgtgttcttctctggctacaccttcaagcacaagatggtgtatgaggacaccctgaccctgttccccttcatgagcatggagaaccctggcctgtgggtgctgggctgccacaacagcgacttcaggaacaggggcatgactgccctgctgaaagtctccagctgtgaccggaacaccggggactactacgaggacacatacgaggacatcccaacttacctgctgagcgaaaacaatgtgatcgagcccaggagcttctctcagaaccccccagtgctgaagaggcaccagagggagatcaccctgaccaccctgcagtctgagcaggaggagatcgactatgatgacaccatcagcattgagacaaagagggaggacttcgacatctacggggaggacgagaaccagggacccaggagcttccagaagaggaccaggcactacttcattgctgctgtggagaggctgtgggactatggcatgtcccgcagcccccatgtgctgaggaacagggcccagtctggcagcgtgccccagttcaagaaagtcgtgttccaggagttcaccgacggcagcttcacccagcccctgtacagaggggagctgaacgagcacctgggcctgctgggcccctacatcagggccgaggtggaggacaacatcatggtgaccttcaagaaccaggccagcaggccctacagcttctacagcagcctgatcagctacgaggaggaccagaggcagggggctgagcccaggaagaactttgtgaagcccaatgaaaccaagacctacttctggaaggtgcagcaccacatggcccccaccaaggacgagttcgactgcaaggcctgggcctacttctctgacgtggacctggagaaggacatgcactctggcctgattggccccctgctgatttgccacaccaacaccctgaaccctgcccatggcaggcaggtgactgtgcaggagttcgccctgttcttcaccatcttcgatgaaaccaagagctggtacttcactgagaacatggagaggaactgcagggccccctgcaacatccagatggaggaccccaccttcaaggagaactacaggttccatgccatcaatggctacgtgatggacaccctgcctggcctggtcatggcccaggaccagaggatcaggtggtatctgctgagcatgggcagcaacgagaacatccacagcatccacttctctggccacgtgttcactgtgaggaagaaggaggagtacaagatggccgtgtacaacctgtaccctggggtgttcgaaaccgtggagatgctgcccagcaaggccggcatctggagggtggagtgcctgattggggagcacctgcacgccggcatgagcaccctgttcctggtgtacagcaaacagtgccagacccccctgggcatggcctctggccacatcagggacttccagatcactgcctctggccagtacggccagtgggcccccaagctggccaggctgcactactccggaagcatcaatgcctggagcaccaaggagcccttcagctggatcaaagtggacctgctggcccccatgatcatccacggcatcaagacccagggggccaggcagaagttctccagcctgtacatcagccagttcatcatcatgtacagcctggacggcaagaagtggcagacctacaggggcaacagcaccggcaccctgatggtgttcttcggcaacgtggacagcagcggcatcaagcacaacatcttcaacccccccatcatcgccagatacatcaggctgcaccccacccactacagcatcaggagcaccctgaggatggagctgatgggctgtgacctgaacagctgcagcatgcccctgggcatggagagcaaggccatctctgacgcccagatcactgcctccagctacttcaccaacatgtttgccacctggagccccagccaggccaggctgcacctgcagggcaggacaaatgcctggaggccccaggtcaacaaccccaaggagtggctgcaggtggacttccagaagaccatgaaggtgactgggatcaccacccagggggtgaagagcctgctgaccagcatgtacgtgaaggagttcctgatctccagcagccaggacggccaccattggaccctgttcctgcagaatggcaaggtgaaggtgttccagggcaaccaggacagcttcacccctgtggtcaacagcctggacccccccctgctgaccagatacctgaggatccacccccagagctgggtgcaccagatcgccctgaggctggaggtgctgggctgtgaggcccagcagctgtactga

SEQ ID NO: 9 - DNA, 4404 bp, Artificial Sequence
  synthetic lcoET3 with CpGs
atgcagctggaactgtctacctgtgtgtttctgtgtctgctgcctctggggttttctgctatccgccgctactatctgggagccgtggagctgtcctgggactacaggcagagcgagctgctgagagaactgcacgtggataccagattcccagctaccgctccaggagctctgcctctgggcccatccgtgctgtacaagaaaaccgtcttcgtggagtttaccgaccagctgttcagcgtggccaggccaagaccaccttggatgggactgctgggaccaaccatccaggctgaggtgtacgataccgtggtcgtgaccctgaaaaacatggcctcccatcccgtgagcctgcacgctgtcggggtgtccttctggaagtccagcgagggagccgagtacgaagaccatacctcccagcgcgagaaagaagacgataaggtgctgcctggcaaaagccagacctatgtctggcaggtgctgaaggagaacggaccaaccgctagcgacccaccatgcctgacctactcttatctgtcccacgtcgatctggtgaaggacctgaattccggactgatcggagctctgctggtgtgtagagagggaagcctgaccagagaaagaacccagaacctgcatgagttcgtcctgctgttcgccgtgtttgacgaagggaagagctggcactctgcccgcaatgactcctggaccagagctatggatccagctcctgctagagctcagcctgctatgcacaccgtcaacggctacgtgaatcggtctctgccaggactgatcggctgccataagaaaagcgtctattggcacgtgatcggaatgggcaccagccccgaggtgcattctatcttcctggaaggccacacctttctggtcaggcaccatagacaggcctctctggagatctcccctctgaccttcctgaccgctcagacctttctgatggacctggggcagttcctgctgttttgccatatctcttcccaccatcacggaggaatggaggctcacgtcagggtggaatcctgtgctgaggaaccacagctgagaagaaaggctgatgaggaagaggactacgacgataacctgtatgacagcgatatggacgtcgtgcgcctggacggcgacgatgtcagccctttcatccagatccggtctgtggccaagaaacatccaaagacctgggtccactacatcgccgctgaagaggaagattgggactatgcccccctggtgctggctcctgacgatagatcctacaaaagccagtatctgaacaatgggccccagcgcatcggacggaagtacaagaaagtgaggttcatggcctataccgacgagacctttaagaccagagaggctatccagcacgaatccgggatcctgggacctctgctgtacggcgaagtgggggataccctgctgatcatcttcaagaaccaggcctccaggccatacaatatctatccccatggcatcaccgacgtgagaccactgtacagcaggagactgcccaagggggtcaaacacctgaaggatttccccatcctgcctggagagatctttaagtataaatggaccgtcaccgtggaagacgggcctaccaagtccgatccacgctgcctgacccggtactatagctctttcgtgaacatggagagagacctggctagcggactgatcggacccctgctgatctgttacaaagagagcgtggaccagaggggcaaccagatcatgtctgataagagaaatgtcatcctgttctccgtgtttgacgagaaccgcagctggtacctgaccgagaacatccagcggttcctgccaaatccagctggagtgcagctggaggacccagaatttcaggcttccaacatcatgcatagcatcaatggctacgtgttcgatagcctgcagctgtctgtctgcctgcacgaggtggcctactggtatatcctgtccatcggcgctcagaccgacttcctgtccgtgttctttagcgggtacacctttaagcataaaatggtgtatgaggataccctgaccctgttccccttttctggcgagaccgtgttcatgtccatggaaaaccctggcctgtggatcctggggtgccacaacagcgacttcaggaatagaggaatgaccgccctgctgaaagtgtccagctgtgataagaataccggcgattactatgaggactcttacgaagatatctccgcttatctgctgagcaagaacaatgccatcgagcccaggtctttcgctcagaactccagacctccaagcgcttctgctcctaagccacctgtgctgagaagacatcagagggacatctccctgcctaccttccagccagaggaagataaaatggactacgacgatatcttcagcaccgagaccaagggggaagattttgacatctatggagaggacgaaaaccaggatccaagatccttccagaagagaaccagacactactttatcgccgctgtggagcagctgtgggactatgggatgtccgaaagcccacgggccctgaggaacagagctcagaatggagaggtgccccgcttcaagaaagtcgtgttccgggagtttgccgacggcagctttacccagccatcttacaggggggagctgaacaagcatctggggctgctgggaccctatatcagagccgaggtcgaagataacatcatggtgaccttcaagaatcaggcttctcgcccctactccttttattcttccctgatctcctaccctgacgatcaggagcagggcgccgaacctaggcacaacttcgtgcagccaaatgagaccagaacctacttttggaaggtgcagcatcacatggctcccaccgaggatgaattcgactgcaaagcttgggcctatttttccgatgtcgacctggagaaggacgtgcatagcggcctgatcgggcctctgctgatctgtcgcgccaacaccctgaatgctgctcacggaagacaggtcaccgtgcaggagttcgctctgttctttaccatctttgacgaaaccaagagctggtacttcaccgagaacgtggaaaggaattgcagagccccctgtcatctgcagatggaggaccctaccctgaaggaaaactacaggttccacgccatcaatggatatgtcatggataccctgcccggcctggtcatggctcagaaccagcgcatccggtggtacctgctgtctatgggatccaacgagaatatccatagcatccacttctctggccatgtcttttccgtgaggaagaaagaggaatacaaaatggccgtgtacaatctgtatcctggggtcttcgagaccgtggaaatgctgccaagcaaagtgggaatctggagaatcgagtgcctgatcggcgaacacctgcaggccgggatgagcaccaccttcctggtgtactctaagaaatgtcagaccccactggggatggcctccggacatatccgcgacttccagatcaccgctagcggacagtacggacagtgggctccaaagctggctagactgcactattctggctccatcaacgcctggtctaccaaagagccattctcctggatcaaggtggacctgctggcccccatgatcatccacggaatcaaaacccagggcgctaggcagaagttcagctctctgtacatctcccagtttatcatcatgtatagcctggacgggaagaaatggcagacctacagaggcaattccaccgggaccctgatggtcttctttggaaacgtggattccagcggcatcaagcacaacatcttcaatccacccatcatcgcccgctacatccggctgcatcctacccactatagcatcaggtctaccctgagaatggagctgatgggatgcgacctgaacagctgttctatgccactgggcatggagtccaaggctatcagcgatgcccagatcaccgcttcttcctacttcaccaatatgtttgctacctggtccccaagcaaggctagactgcacctgcagggaagatccaacgcttggagaccccaggtgaacaatcctaaggagtggctgcaggtcgacttccagaaaaccatgaaggtcaccggggtgaccacccagggagtgaaatctctgctgacctccatgtacgtcaaggagttcctgatcagctcttcccaggacggccaccagtggaccctgttctttcagaacggcaaggtcaaagtgttccaggggaatcaggactcttttacccccgtcgtgaactccctggatcctccactgctgaccaggtacctgagaatccatcctcagagctgggtgcaccagatcgctctgagaatggaggtcctgggatgcgaagctcaggacctgtattga

SEQ ID NO: 10 - DNA, 4403 bp, Artificial Sequence
  synthetic lcoET3 CpGs removed
atgcagctggaactgtctacctgtgtgtttctgtgtctgctgcctctggggttttctgctatcaggagatactatctgggagctgtggagctgtcctgggactacaggcagtctgagctgctgagagaactgcatgtggataccagattcccagctacagctccaggagctctgcctctgggcccatctgtgctgtacaagaaaacagtctttgtggagtttacagaccagctgttctctgtggccaggccaagaccaccttggatgggactgctgggaccaaccatccaggctgaggtgtatgatacagtggtggtgaccctgaaaaacatggcctcccatcctgtgagcctgcatgctgtgggggtgtccttctggaagtcctctgagggagctgagtatgaagaccatacctcccagagggagaaagaagatgataaggtgctgcctggcaaaagccagacctatgtctggcaggtgctgaaggagaatggaccaactgcttctgacccaccatgcctgacctactcttatctgtcccatgtggatctggtgaaggacctgaattctggactgattggagctctgctggtgtgtagagagggaagcctgaccagagaaagaacccagaacctgcatgagtttgtcctgctgtttgctgtgtttgatgaagggaagagctggcactctgccaggaatgactcctggaccagagctatggatccagctcctgctagagctcagcctgctatgcacacagtcaatggctatgtgaataggtctctgccaggactgattggctgccataagaaatctgtctattggcatgtgattggaatgggcaccagccctgaggtgcattctatcttcctggaaggccacacctttctggtcaggcaccatagacaggcctctctggagatctcccctctgaccttcctgacagctcagacctttctgatggacctggggcagttcctgctgttttgccatatctcttcccaccatcatggaggaatggaggctcatgtcagggtggaatcctgtgctgaggaaccacagctgagaagaaaggctgatgaggaagaggactatgatgataacctgtatgactctgatatggatgtggtgaggctggatggggatgatgtcagccctttcatccagatcaggtctgtggccaagaaacatccaaagacctgggtccactacattgctgctgaagaggaagattgggactatgcccccctggtgctggctcctgatgatagatcctacaaaagccagtatctgaacaatgggccccagaggattggaaggaagtacaagaaagtgaggttcatggcctatacagatgagacctttaagaccagagaggctatccagcatgaatctgggatcctgggacctctgctgtatggagaagtgggggatacctgctgatcatcttcaagaaccaggcctccaggccatacaatatctatccccatggcatcacagatgtgagaccactgtacagcaggagactgcccaagggggtcaaacacctgaaggatttccccatcctgcctggagagatctttaagtataaatggacagtcacagtggaagatgggcctaccaagtctgatccaaggtgcctgaccagatactatagctcttttgtgaacatggagagagacctggcttctggactgattggacccctgctgatctgttacaaagagtctgtggaccagaggggcaaccagatcatgtctgataagagaaatgtcatcctgttctctgtgtttgatgagaacaggagctggtacctgacagagaacatccagaggttcctgccaaatccagctggagtgcagctggaggacccagaatttcaggcttccaacatcatgcatagcatcaatggctatgtgtttgatagcctgcagctgtctgtctgcctgcatgaggtggcctactggtatatcctgtccattggagctcagacagacttcctgtctgtgttctttagtgggtacacctttaagcataaaatggtgtatgaggataccctgaccctgttccccttttctggggagacagtgttcatgtccatggaaaaccctggcctgtggatcctggggtgccacaactctgacttcaggaatagaggaatgacagccctgctgaaagtgtccagctgtgataagaatacaggggattactatgaggactcttatgaagatatctctgcttatctgctgagcaagaacaatgccattgagcccaggtcttttgctcagaactccagacctccatctgcttctgctcctaagccacctgtgctgagaagacatcagagggacatctccctgcctaccttccagccagaggaagataaaatggactatgatgatatcttcagcacagagaccaagggggaagattttgacatctatggagaggatgaaaaccaggatccaagatccttccagaagagaaccagacactactttattgctgctgtggagcagctgtgggactatgggatgtctgaaagcccaagggccctgaggaacagagctcagaatggagaggtgcccagattcaagaaagtggtgttcagagagtttgctgatggcagctttacccagccatcttacaggggggagctgaacaagcatctggggctgctgggaccctatatcagagctgaggtggaagataacatcatggtgaccttcaagaatcaggcttctaggccctactccttttattcttccctgatctcctaccctgatgatcaggagcagggagctgaacctaggcacaactttgtgcagccaaatgagaccagaacctacttttggaaggtgcagcatcacatggctcccacagaggatgaatttgactgcaaagcttgggcctatttttctgatgtggacctggagaaggatgtgcattctggcctgattgggcctctgctgatctgtagggccaacaccctgaatgctgctcatggaagacaggtcacagtgcaggagtttgctctgttctttaccatctttgatgaaaccaagagctggtacttcacagagaatgtggaaaggaattgcagagccccctgtcatctgcagatggaggaccctaccctgaaggaaaactacaggttccatgccatcaatggatatgtcatggataccctgcctggcctggtcatggctcagaaccagaggatcagatggtacctgctgtctatgggatccaatgagaatatccatagcatccacttctctggccatgtcttttctgtgaggaagaaagaggaatacaaaatggctgtgtacaatctgtatcctggggtctttgagacagtggaaatgctgccaagcaaagtgggaatctggagaattgagtgcctgattggggaacacctgcaggctgggatgagcaccaccttcctggtgtactctaagaaatgtcagaccccactggggatggcctctggacatatcagggacttccagatcacagcttctggacagtatggacagtgggctccaaagctggctagactgcactattctggctccatcaatgcctggtctaccaaagagccattctcctggatcaaggtggacctgctggcccccatgatcatccatggaatcaaaacccagggagctaggcagaagttcagctctctgtacatctcccagtttatcatcatgtatagcctggatgggaagaaatggcagacctacagaggcaattccactgggaccctgatggtcttctttggaaatgtggattcctctggcatcaagcacaacatcttcaatccacccatcattgccaggtacatcaggctgcatcctacccactatagcatcaggtctaccctgagaatggagctgatgggatgtgacctgaacagctgttctatgccactgggcatggagtccaaggctatctctgatgcccagatcacagcttcttcctacttcaccaatatgtttgctacctggtccccaagcaaggctagactgcacctgcagggaagatccaatgcttggagaccccaggtgaacaatcctaaggagtggctgcaggtggacttccagaaaaccatgaaggtcacaggggtgaccacccagggagtgaaatctctgctgacctccatgtatgtcaaggagttcctgatcagctcttcccaggatggccaccagtggaccctgttctttcagaatggcaaggtcaaagtgttccaggggaatcaggactcttttaccccagtggtgaactccctggatcctccactgctgaccaggtacctgagaatccatcctcagagctgggtgcaccagattgctctgagaatggaggtcctgggatgtgaagctcaggacctgtattga

SEQ ID NO: 11 - DNA, 4404 bp, Artificial Sequence
  synthetic NoCoET3
atgcagctagagctctccacctgtgtctttctgtgtctcttgccactcggctttagtgccatcaggagatactacctgggcgcagtggaactgtcctgggactaccggcaaagtgaactcctccgtgagctgcacgtggacaccagatttcctgctacagcgccaggagctcttccgttgggcccgtcagtcctgtacaaaaagactgtgttcgtagagttcacggatcaacttttcagcgttgccaggcccaggccaccatggatgggtctgctgggtcctaccatccaggctgaggtttacgacacggtggtcgttaccctgaagaacatggcttctcatcccgttagtcttcacgctgtcggcgtctccttctggaaatcttccgaaggcgctgaatatgaggatcacaccagccaaagggagaaggaagacgataaagtccttcccggtaaaagccaaacctacgtctggcaggtcctgaaagaaaatggtccaacagcctctgacccaccatgtcttacctactcatacctgtctcacgtggacctggtgaaagacctgaattcgggcctcattggagccctgctggtttgtagagaagggagtctgaccagagaaaggacccagaacctgcacgaatttgtactactttttgctgtctttgatgaagggaaaagttggcactcagcaagaaatgactcctggacacgggccatggatcccgcacctgccagggcccagcctgcaatgcacacagtcaatggctatgtcaacaggtctctgccaggtctgatcggatgtcataagaaatcagtctactggcacgtgattggaatgggcaccagcccggaagtgcactccatttttcttgaaggccacacgtttctcgtgaggcaccatcgccaggcttccttggagatctcgccactaactttcctcactgctcagacattcctgatggaccttggccagttcctactgttttgtcatatctcttcccaccaccatggtggcatggaggctcacgtcagagtagaaagctgcgccgaggagccccagctgcggaggaaagctgatgaagaggaagattatgatgacaatttgtacgactcggacatggacgtggtccggctcgatggtgacgacgtgtctccctttatccaaatccgctcagttgccaagaagcatcctaaaacttgggtacattacattgctgctgaagaggaggactgggactatgctcccttagtcctcgcccccgatgacagaagttataaaagtcaatatttgaacaatggccctcagcggattggtaggaagtacaaaaaagtccgatttatggcatacacagatgaaacctttaagacgcgtgaagctattcagcatgaatcaggaatcttgggacctttactttatggggaagttggagacacactgttgattatatttaagaatcaagcaagcagaccatataacatctaccctcacggaatcactgatgtccgtcctttgtattcaaggagattaccaaaaggtgtaaaacatttgaaggattttccaattctgccaggagaaatattcaaatataaatggacagtgactgtagaagatgggccaactaaatcagatccgcggtgcctgacccgctattactctagtttcgttaatatggagagagatctagcttcaggactcattggccctctcctcatctgctacaaagaatctgtagatcaaagaggaaaccagataatgtcagacaagaggaatgtcatcctgttttctgtatttgatgagaaccgaagctggtacctcacagagaatatacaacgctttctccccaatccagctggagtgcagcttgaggatccagagttccaagcctccaacatcatgcacagcatcaatggctatgtttttgatagtttgcagttgtcagtttgtttgcatgaggtggcatactggtacattctaagcattggagcacagactgacttcctttctgtcttcttctctggatataccttcaaacacaaaatggtctatgaagacacactcaccctattcccattctcaggagaaactgtcttcatgtcgatggaaaacccaggtctatggattctggggtgccacaactcagactttcggaacagaggcatgaccgccttactgaaggtttctagttgtgacaagaacactggtgattattacgaggacagttatgaagatatttcagcatacttgctgagtaaaaacaatgccattgaacctaggagctttgcccagaattcaagaccccctagtgcgagcgctccaaagcctccggtcctgcgacggcatcagagggacataagccttcctacttttcagccggaggaagacaaaatggactatgatgatatcttctcaactgaaacgaagggagaagattttgacatttacggtgaggatgaaaatcaggaccctcgcagctttcagaagagaacccgacactatttcattgctgcggtggagcagctctgggattacgggatgagcgaatccccccgggcgctaagaaacagggctcagaacggagaggtgcctcggttcaagaaggtggtcttccgggaatttgctgacggctccttcacgcagccgtcgtaccgcggggaactcaacaaacacttggggctcttgggaccctacatcagagcggaagttgaagacaacatcatggtaactttcaaaaaccaggcgtctcgtccctattccttctactcgagccttatttcttatccggatgatcaggagcaaggggcagaacctcgacacaacttcgtccagccaaatgaaaccagaacttacttttggaaagtgcagcatcacatggcacccacagaagacgagtttgactgcaaagcctgggcctacttttctgatgttgacctggaaaaagatgtgcactcaggcttgatcggcccccttctgatctgccgcgccaacaccctgaacgctgctcacggtagacaagtgaccgtgcaagaatttgctctgtttttcactatttttgatgagacaaagagctggtacttcactgaaaatgtggaaaggaactgccgggccccctgccatctgcagatggaggaccccactctgaaagaaaactatcgcttccatgcaatcaatggctatgtgatggatacactccctggcttagtaatggctcagaatcaaaggatccgatggtatctgctcagcatgggcagcaatgaaaatatccattcgattcattttagcggacacgtgttcagtgtacggaaaaaggaggagtataaaatggccgtgtacaatctctatccgggtgtctttgagacagtggaaatgctaccgtccaaagttggaatttggcgaatagaatgcctgattggcgagcacctgcaagctgggatgagcacgactttcctggtgtacagcaagaagtgtcagactcccctgggaatggcttctggacacattagagattttcagattacagcttcaggacaatatggacagtgggccccaaagctggccagacttcattattccggatcaatcaatgcctggagcaccaaggagcccttttcttggatcaaggtggatctgttggcaccaatgattattcacggcatcaagacccagggtgcccgtcagaagttctccagcctctacatctctcagtttatcatcatgtatagtcttgatgggaagaagtggcagacttatcgaggaaattccactggaaccttaatggtcttctttggcaatgtggattcatctgggataaaacacaatatttttaaccctccaattattgctcgatacatccgtttgcacccaactcattatagcattcgcagcactcttcgcatggagttgatgggctgtgatttaaatagttgcagcatgccattgggaatggagagtaaagcaatatcagatgcacagattactgcttcatcctactttaccaatatgtttgccacctggtctccttcaaaagctcgacttcacctccaagggaggagtaatgcctggagacctcaggtgaataatccaaaagagtggctgcaagtggacttccagaagacaatgaaagtcacaggagtaactactcagggagtaaaatctctgcttaccagcatgtatgtgaaggagttcctcatctccagcagtcaagatggccatcagtggactctcttttttcagaatggcaaagtaaaggtttttcagggaaatcaagactccttcacacctgtggtgaactctctagacccaccgttactgactcgctaccttcgaattcacccccagagttgggtgcaccagattgccctgaggatggaggttctgggctgcgaggcacaggacctctactga

SEQ ID NO: 12 - DNA, 4404 bp, Artificial Sequence
  synthetic mcoET3
atgcagctggagctctcaacctgtgtgttcctctgcctgctccccctgggattttcagctatcaggagatactatctgggagcagtggaactgtcctgggactacaggcagtcagagctgctcagagaactgcatgtggatactaggttccctgcaacagctcctggagcactgccactgggaccttcagtgctgtacaagaaaactgtctttgtggagtttacagaccagctgttcagtgtggccaggcccaggcccccctggatggggctgctgggacccaccatccaggctgaagtgtatgatactgtggtggtgaccctgaaaaacatggcctctcatccagtcagcctgcatgctgtgggagtgagcttctggaagagcagtgagggagctgagtatgaagaccatacctcacagagggagaaagaagatgataaggtgctgccaggaaaaagccagacctatgtgtggcaggtgctgaaggagaatggccctacagcttcagatcctccctgcctcacatactcttatctgagccatgtggatctggtgaaggacctcaatagtggcctgattggggcactgctggtgtgcagagaggggtccctcacaagggaaagaactcagaacctgcatgagtttgtcctgctctttgctgtgtttgatgagggaaagtcctggcactcagcaaggaatgacagctggaccagggctatggacccagcaccagccagagctcagccagctatgcacactgtcaatggctatgtgaataggtccctgcctggactcattggctgccataagaaatcagtctattggcatgtgattggaatgggcaccagcccagaggtgcattccatcttcctggaaggccacacatttctggtcaggcaccatagacaggccagcctggagatcagcccactgactttcctcacagcacagacatttctgatggacctggggcagttcctgctcttttgccatatctcaagtcaccatcatggagggatggaggctcatgtcagggtggaaagctgtgcagaggaacctcagctgaggaggaaggcagatgaggaagaggactatgatgataacctgtatgactcagatatggatgtggtgaggctggatggagatgatgtcagcccattcatccagatcaggtcagtggctaagaaacaccctaagacctgggtccactacattgcagctgaagaggaagattgggactatgcacccctggtgctggccccagatgatagaagttacaaatctcagtatctgaacaatgggccccagaggattggaaggaagtacaagaaagtgaggttcatggcttatactgatgagacctttaagacaagagaggcaatccagcatgaaagtggcatcctgggaccactgctctatggagaagtgggggataccctgctcatcatcttcaagaaccaggcctcaaggccttacaatatctatccccatggcatcacagatgtgaggcctctctacagcaggagactgcccaagggagtcaaacacctcaaggatttccccatcctgccaggggaaatcttcaagtataaatggacagtcactgtggaagatgggccaactaagtcagatcctaggtgcctgaccaggtactattctagctttgtgaacatggagagggacctggcttcaggactgattggacctctgctcatctgctacaaagaatcagtggaccagaggggcaaccagatcatgagtgataagagaaatgtcatcctgttctcagtgtttgatgagaataggagttggtatctgacagaaaacatccagaggttcctgcctaatcctgcaggagtgcagctggaggacccagaatttcaggcttcaaacatcatgcatagtatcaatggctatgtgtttgatagtctgcagctctctgtctgcctgcatgaggtggcctactggtatatcctcagcattggagctcagactgacttcctgagtgtgttcttttcaggctacacattcaagcataagatggtctatgaagataccctgacactcttccccttttctggggagactgtgtttatgagcatggaaaacccaggcctgtggattctggggtgccacaacagtgacttcaggaatagagggatgactgctctgctcaaagtgtcctcatgtgataagaatactggagattactatgaggactcttatgaagatatcagtgcatatctgctctccaaaaacaatgccattgagcccaggtcatttgctcagaacagtagaccaccttctgcaagtgcaccaaagcctccagtgctgaggagacaccagagggacatcagcctgccaaccttccagcctgaggaagataaaatggactatgatgatatcttctccactgagaccaagggggaagattttgacatctatggagaggatgaaaaccaggaccccaggtccttccagaagaggaccagacactactttattgcagctgtggagcagctgtgggactatggcatgtctgaatcacctagagctctgaggaacagagcacagaatggggaggtgcccaggttcaagaaagtggtgttcagagaatttgcagatggctcttttacccagcctagctacaggggggagctcaacaagcatctggggctgctgggaccctatatcagagcagaggtggaagataacatcatggtgacattcaagaatcaggcctcaagaccctacagtttttatagttctctgatcagctacccagatgatcaggagcagggggctgaaccaaggcacaactttgtgcagcctaatgagacaagaacttacttttggaaggtccagcatcacatggctcccacagaggatgagtttgactgcaaggcctgggcatatttttctgatgtggacctggagaaggatgtgcatagtggcctcattgggccactgctcatctgcagggcaaacacactgaatgctgcacatggcaggcaggtcactgtgcaggagtttgccctgttctttacaatctttgatgaaactaagtcctggtacttcacagagaatgtggaaaggaattgcagagccccctgccatctccagatggaggacccaactctgaaggaaaactacaggttccatgctatcaatggatatgtcatggatacactgccaggcctggtgatggcacagaaccagaggatcaggtggtatctgctcagcatggggtccaatgagaatatccattctatccacttctcaggacatgtcttttcagtgaggaagaaagaggaatataaaatggctgtgtacaatctgtatccaggggtctttgagacagtggaaatgctgcctagcaaagtggggatctggagaattgagtgcctcattggagaacacctgcaggcagggatgtccaccacatttctggtgtactcaaagaaatgccagactcccctggggatggcaagtggacatatcagggacttccagatcactgcatcaggacagtatggacagtgggcaccaaagctggctaggctccactatagtggctctatcaatgcttggagtaccaaagagcctttctcttggatcaaggtggatctgctggcccccatgatcatccatggaatcaaaacacagggagctagacagaagttcagctccctgtacatcagtcagtttatcatcatgtattctctggatgggaagaaatggcagacctacaggggcaatagcactgggacactgatggtcttctttggaaatgtggattcaagtggcatcaagcacaacatcttcaatcctcccatcattgccaggtacatcagactgcatcccacacactattcaatcaggagtactctcagaatggagctgatggggtgtgacctcaacagctgctccatgccactgggaatggaatccaaggcaatctcagatgcccagatcactgcttctagctacttcaccaatatgtttgcaacatggtcacccagtaaagcaaggctgcacctccagggaaggtccaatgcttggagaccccaggtgaacaatccaaaggagtggctgcaggtggactttcagaaaaccatgaaggtcacaggggtgactacccagggagtgaaaagtctgctcacctctatgtatgtcaaggagttcctgatctcctcaagtcaggatggccaccagtggacactgttctttcagaatggcaaggtcaaagtgttccaggggaatcaggacagctttacaccagtggtgaacagcctggacccccctctgctcactagatatctgagaatccatccacagagctgggtgcaccagattgcactcagaatggaggtcctgggctgtgaagcccaggacctgtattga

SEQ ID NO: 13 - DNA, 4374 bp, Artificial Sequence
  synthetic lcoHSQ with CpGs
atgcagatcgaactgtctacctgtttctttctgtgcctgctgcggttttgtttttccgctaccagaagatactacctgggagccgtcgaactgagctgggattacatgcagtctgacctgggagagctgcccgtggacgctagattcccacctagagtccctaagtccttccccttcaacaccagcgtggtctacaagaaaaccctgttcgtggagtttaccgaccacctgttcaacatcgctaagcctagaccaccatggatgggactgctgggaccaaccatccaggccgaggtgtacgacaccgtggtcatcaccctgaaaaacatggcttctcaccccgtgtccctgcatgctgtgggcgtctcctactggaaggccagcgaaggggctgagtatgacgatcagaccagccagcgggaaaaagaggacgataaggtgttccctggcgggtcccatacctacgtgtggcaggtcctgaaggagaatggaccaatggcttccgaccctctgtgcctgacctactcttatctgtcccacgtggacctggtcaaggatctgaacagcggcctgatcggggctctgctggtgtgtcgcgaagggtccctggccaaggagaaaacccagaccctgcataagttcatcctgctgttcgccgtgtttgacgaaggaaaaagctggcactctgagaccaagaactctctgatgcaggacagggatgccgcttccgccagagcttggcccaagatgcacaccgtgaacggctacgtcaataggagcctgcctggactgatcggctgccacagaaagtccgtgtattggcatgtcatcggaatgggcaccacccctgaagtgcacagcatcttcctggaggggcatacctttctggtccgcaaccaccggcaggctagcctggagatctctccaatcaccttcctgaccgcccagaccctgctgatggacctgggacagttcctgctgttttgccacatctccagccaccagcatgatggcatggaggcttacgtgaaagtcgactcctgtcccgaggaacctcagctgaggatgaagaacaatgaggaagccgaagactatgacgatgacctgaccgacagcgagatggatgtggtccgcttcgatgacgataactctccctcctttatccagatccggtccgtggccaagaaacaccctaagacctgggtccattacatcgccgctgaggaagaggactgggattatgctccactggtgctggcccccgacgatagatcctacaaaagccagtatctgaacaatggaccccagaggatcggcagaaagtacaagaaagtgaggttcatggcttataccgatgagacctttaagaccagagaagccatccagcacgagtccgggatcctgggacctctgctgtacggcgaagtgggggacaccctgctgatcatcttcaagaaccaggccagcaggccttacaatatctatccacatggcatcaccgatgtgagacctctgtactcccgccggctgccaaagggcgtgaaacacctgaaggacttcccaatcctgcccggggaaatctttaagtataaatggaccgtcaccgtcgaggatgggcccaccaagagcgaccctaggtgcctgaccagatactattcttccttcgtgaatatggagagagacctggcttccggactgatcggacccctgctgatctgttacaaagagagcgtggatcagcgcggcaaccagatcatgtctgacaagcggaatgtgatcctgttcagcgtctttgacgaaaaccgctcttggtacctgaccgagaacatccagcggttcctgcctaatccagctggagtgcagctggaagatcccgagttccaggcctctaacatcatgcattccatcaatggctacgtgttcgactccctgcagctgagcgtgtgcctgcacgaggtcgcttactggtatatcctgagcatcggagcccagaccgatttcctgtctgtgttcttttccggctacacctttaagcataaaatggtgtatgaggacaccctgaccctgttcccattttccggcgaaaccgtgttcatgagcatggagaatcccgggctgtggatcctgggatgccacaactccgatttcaggaatagagggatgaccgccctgctgaaagtgagctcttgtgacaagaacaccggagactactatgaagatagctacgaggacatctctgcttatctgctgtccaaaaacaatgccatcgagcccaggagcttctctcagaaccctccagtgctgaagcgccaccagcgggagatcaccagaaccaccctgcagagcgatcaggaagagatcgactacgacgataccatctccgtggaaatgaagaaagaggacttcgatatctatgacgaagatgagaaccagtctcccaggtccttccagaagaaaaccagacattactttatcgccgctgtggagcggctgtgggactatggcatgtccagctctcctcacgtgctgagaaatagagctcagtccggaagcgtcccacagttcaagaaagtggtcttccaggagtttaccgacggaagctttacccagccactgtaccgcggcgaactgaacgagcacctggggctgctgggaccctatatccgggctgaagtggaggataacatcatggtcaccttcaggaatcaggccagcagaccctactctttttattccagcctgatctcctacgaagaggaccagagacagggagctgaaccaagaaaaaacttcgtgaagcctaatgagaccaaaacctacttttggaaggtgcagcaccatatggcccctaccaaagacgagttcgattgcaaggcctgggcttattttagcgacgtggatctggagaaggacgtccactccggcctgatcgggccactgctggtgtgtcataccaacaccctgaatccagctcacggaaggcaggtgaccgtccaggaattcgccctgttctttaccatctttgatgagaccaagagctggtacttcaccgaaaacatggagaggaattgcagagccccatgtaacatccagatggaagaccccaccttcaaggagaactacagatttcatgctatcaatgggtatatcatggataccctgccaggactggtcatggctcaggaccagaggatcagatggtacctgctgagcatggggtctaacgagaatatccactccatccatttcagcggacacgtgtttaccgtccgcaagaaagaagagtacaagatggccctgtacaacctgtatcccggcgtgttcgaaaccgtcgagatgctgccttccaaggctgggatctggcgggtggaatgcctgatcggggagcacctgcatgccggaatgtctaccctgttcctggtgtactccaataagtgtcagacccccctggggatggctagcggacatatccgcgacttccagatcaccgcttccggacagtacggacagtgggctcctaagctggctagactgcactattctggctccatcaacgcttggtctaccaaagagcctttctcctggatcaaggtggacctgctggctccaatgatcatccatggcatcaaaacccagggggccaggcagaagttctcttccctgtacatcagccagtttatcatcatgtattctctggatgggaagaaatggcagacctacagaggcaattccaccgggaccctgatggtgttctttggcaacgtcgacagctctgggatcaagcacaacatcttcaatccccctatcatcgcccgctacatccggctgcacccaacccattattccatccgcagcaccctgcggatggagctgatggggtgcgatctgaacagctgttctatgcccctgggaatggagtctaaggccatctccgacgctcagatcaccgcctccagctacttcaccaatatgtttgctacctggtccccaagcaaggctagactgcatctgcagggaagaagcaacgcttggagaccacaggtgaacaatcccaaggagtggctgcaggtcgacttccagaaaaccatgaaggtgaccggagtcaccacccagggcgtgaaaagcctgctgacctctatgtacgtcaaggagttcctgatctcttccagccaggacgggcaccagtggaccctgttctttcagaacggaaaggtgaaagtcttccagggcaatcaggattcctttacccctgtggtcaacagcctggacccacccctgctgaccaggtacctgagaatccacccacagtcctgggtgcatcagatcgctctgaggatggaagtcctgggctgcgaggcccaggacctgtattga

SEQ ID NO: 14 - DNA, 4374 bp, Artificial Sequence
  synthetic lcoHSQ CpGs removed
atgcagattgaactgtctacctgtttctttctgtgcctgctgaggttttgtttttctgctaccagaagatactacctgggagctgtggaactgagctgggattacatgcagtctgacctgggagagctgcctgtggatgctagattcccacctagagtccctaagtccttccccttcaacacctctgtggtctacaagaaaaccctgtttgtggagtttacagaccacctgttcaacattgctaagcctagaccaccatggatgggactgctgggaccaaccatccaggcagaggtgtatgacacagtggtcatcaccctgaaaaacatggcttctcaccctgtgtccctgcatgctgtgggagtctcctactggaaggcctctgaaggggctgagtatgatgatcagaccagccagagggaaaaagaggatgataaggtgttccctggagggtcccatacctatgtgtggcaggtcctgaaggagaatggaccaatggcttctgaccctctgtgcctgacctactcttatctgtcccatgtggacctggtcaaggatctgaactctggcctgattggggctctgctggtgtgtagggaagggtccctggccaaggagaaaacccagaccctgcataagttcatcctgctgtttgctgtgtttgatgaaggaaaaagctggcactctgagaccaagaactctctgatgcaggacagggatgctgcttctgccagagcttggcccaagatgcacacagtgaatggctatgtcaataggagcctgcctggactgattggctgccacagaaagtctgtgtattggcatgtcattggaatgggcaccacccctgaagtgcacagcatcttcctggaggggcatacctttctggtcaggaaccacaggcaggctagcctggagatctctccaatcaccttcctgacagcccagaccctgctgatggacctgggacagttcctgctgttttgccacatctccagccaccagcatgatggcatggaggcttatgtgaaagtggactcctgtcctgaggaacctcagctgaggatgaagaacaatgaggaagctgaagactatgatgatgacctgacagactctgagatggatgtggtcaggtttgatgatgataactctccctcctttatccagatcaggtctgtggccaagaaacaccctaagacctgggtccattacattgctgctgaggaagaggactgggattatgctccactggtgctggcccctgatgatagatcctacaaaagccagtatctgaacaatggaccccagaggattggcagaaagtacaagaaagtgaggttcatggcttatacagatgagacctttaagaccagagaagccatccagcatgagtctgggatcctgggacctctgctgtatggggaagtgggggacaccctgctgatcatcttcaagaaccaggccagcaggccttacaatatctatccacatggcatcacagatgtgagacctctgtactccaggaggctgccaaagggggtgaaacacctgaaggacttcccaatcctgcctggggaaatctttaagtataaatggacagtcacagtggaggatgggcccaccaagtctgaccctaggtgcctgaccagatactattcttcctttgtgaatatggagagagacctggcttctggactgattggacccctgctgatctgttacaaagagtctgtggatcagaggggcaaccagatcatgtctgacaagaggaatgtgatcctgttctctgtctttgatgaaaacaggtcttggtacctgacagagaacatccagaggttcctgcctaatccagctggagtgcagctggaagatcctgagttccaggcctctaacatcatgcattccatcaatggctatgtgtttgactccctgcagctgtctgtgtgcctgcatgaggtggcttactggtatatcctgagcattggagcccagacagatttcctgtctgtgttcttttctggctacacctttaagcataaaatggtgtatgaggacaccctgaccctgttcccattttctggagaaactgtgttcatgagcatggagaatcctgggctgtggatcctgggatgccacaactctgatttcaggaatagagggatgacagccctgctgaaagtgagctcttgtgacaagaacacaggagactactatgaagatagctatgaggacatctctgcttatctgctgtccaaaaacaatgccattgagcccaggagcttctctcagaaccctccagtgctgaagaggcaccagagggagatcaccagaaccaccctgcagtctgatcaggaagagattgactatgatgataccatctctgtggaaatgaagaaagaggactttgatatctatgatgaagatgagaaccagtctcccaggtccttccagaagaaaaccagacattactttattgctgctgtggagaggctgtgggactatggcatgtccagctctcctcatgtgctgagaaatagagctcagtctggatctgtcccacagttcaagaaagtggtcttccaggagtttacagatggaagctttacccagccactgtacaggggagaactgaatgagcacctggggctgctgggaccctatatcagggctgaagtggaggataacatcatggtcaccttcaggaatcaggccagcagaccctactctttttattccagcctgatctcctatgaagaggaccagagacagggagctgaaccaagaaaaaactttgtgaagcctaatgagaccaaaacctacttttggaaggtgcagcaccatatggcccctaccaaagatgagtttgattgcaaggcctgggcttatttttctgatgtggatctggagaaggatgtccactctggcctgattgggccactgctggtgtgtcataccaacaccctgaatccagctcatggaaggcaggtgacagtccaggaatttgccctgttctttaccatctttgatgagaccaagagctggtacttcacagaaaacatggagaggaattgcagagccccatgtaacatccagatggaagaccccaccttcaaggagaactacagatttcatgctatcaatgggtatatcatggataccctgccaggactggtcatggctcaggaccagaggatcagatggtacctgctgagcatggggtctaatgagaatatccactccatccatttctctggacatgtgtttacagtaaggaagaaagaagagtacaagatggccctgtacaacctgtatcctggggtgtttgaaacagtggagatgctgccttccaaggctgggatctggagggtggaatgcctgattggggagcacctgcatgctggaatgtctaccctgttcctggtgtactccaataagtgtcagacccccctggggatggcttctggacatatcagggacttccagatcacagcttctggacagtatggacagtgggctcctaagctggctagactgcactattctggctccatcaatgcttggtctaccaaagagcctttctcctggatcaaggtggacctgctggctccaatgatcatccatggcatcaaaacccagggggccaggcagaagttctcttccctgtacatcagccagtttatcatcatgtattctctggatgggaagaaatggcagacctacagaggcaattccacagggaccctgatggtgttctttggcaatgtggacagctctgggatcaagcacaacatcttcaatccccctatcattgccaggtacatcagactgcacccaacccattattccatcaggagcaccctgagaatggagctgatggggtgtgatctgaacagctgttctatgcccctgggaatggagtctaaggccatctctgatgctcagatcacagcctccagctacttcaccaatatgtttgctacctggtccccaagcaaggctagactgcatctgcagggaagaagcaatgcttggagaccacaggtgaacaatcccaaggagtggctgcaggtggacttccagaaaaccatgaaggtgacaggagtcaccacccagggagtgaaaagcctgctgacctctatgtatgtcaaggagttcctgatctcttccagccaggatgggcaccagtggaccctgttctttcagaatggaaaggtgaaagtcttccagggcaatcaggattcctttacccctgtggtcaacagcctggacccacccctgctgaccaggtacctgagaatccacccacagtcctgggtgcatcagattgctctgaggatggaagtcctgggctgtgaggcccaggacctgtattga

SEQ ID NO: 15 - DNA, 4374 bp, Artificial Sequence
  synthetic NoCoHSQ
atgcaaatagagctctccacctgcttctttctgtgccttttgcgattctgctttagtgccaccagaagatactacctgggtgcagtggaactgtcatgggactatatgcaaagtgatctcggtgagctgcctgtggacgcaagatttcctcctagagtgccaaaatcttttccattcaacacctcagtcgtgtacaaaaagactctgtttgtagaattcacggaccaccttttcaacatcgctaagccaaggccaccctggatgggtctgctaggtcctaccatccaggctgaggtttatgatacagtggtcattacacttaagaacatggcttcccatcctgtcagtcttcatgctgttggtgtatcctactggaaagcttctgagggagctgaatatgatgatcagaccagtcaaagggagaaagaagatgataaagtcttccctggtggaagccatacatatgtctggcaggtcctgaaagagaatggtccaatggcctctgacccactgtgccttacctactcatatctttctcatgtggacctggtaaaagacttgaattcaggcctcattggagccctactagtatgtagagaagggagtctggccaaggaaaagacacagaccttgcacaaatttatactactttttgctgtatttgatgaagggaaaagttggcactcagaaacaaagaactccttgatgcaggatagggatgctgcatctgctcgggcctggcctaaaatgcacacagtcaatggttatgtaaacaggtctctgccaggtctgattggatgccacaggaaatcagtctattggcatgtgattggaatgggcaccactcctgaagtgcactcaatattcctcgaaggtcacacatttcttgtgaggaaccatcgccaggcgtccttggaaatctcgccaataactttccttactgctcaaacactcttgatggaccttggacagtttctactgttttgtcatatctcttcccaccaacatgatggcatggaagcttatgtcaaagtagacagctgtccagaggaaccccaactacgaatgaaaaataatgaagaagcggaagactatgatgatgatcttactgattctgaaatggatgtggtcaggtttgatgatgacaactctccttcctttatccaaattcgctcagttgccaagaagcatcctaaaacttgggtacattacattgctgctgaagaggaggactgggactatgctcccttagtcctcgcccccgatgacagaagttataaaagtcaatatttgaacaatggccctcagcggattggtaggaagtacaaaaaagtccgatttatggcatacacagatgaaacctttaagacgcgtgaagctattcagcatgaatcaggaatcttgggacctttactttatggggaagttggagacacactgttgattatatttaagaatcaagcaagcagaccatataacatctaccctcacggaatcactgatgtccgtcctttgtattcaaggagattaccaaaaggtgtaaaacatttgaaggattttccaattctgccaggagaaatattcaaatataaatggacagtgactgtagaagatgggccaactaaatcagatccgcggtgcctgacccgctattactctagtttcgttaatatggagagagatctagcttcaggactcattggccctctcctcatctgctacaaagaatctgtagatcaaagaggaaaccagataatgtcagacaagaggaatgtcatcctgttttctgtatttgatgagaaccgaagctggtacctcacagagaatatacaacgctttctccccaatccagctggagtgcagcttgaggatccagagttccaagcctccaacatcatgcacagcatcaatggctatgtttttgatagtttgcagttgtcagtttgtttgcatgaggtggcatactggtacattctaagcattggagcacagactgacttcctttctgtcttcttctctggatataccttcaaacacaaaatggtctatgaagacacactcaccctattcccattctcaggagaaactgtcttcatgtcgatggaaaacccaggtctatggattctggggtgccacaactcagactttcggaacagaggcatgaccgccttactgaaggtttctagttgtgacaagaacactggtgattattacgaggacagttatgaagatatttcagcatacttgctgagtaaaaacaatgccattgaacctaggagcttctctcagaatccaccagtcttgaaacgccatcaacgggaaataactcgtactactcttcagtcagatcaagaggaaattgactatgatgataccatatcagttgaaatgaagaaggaagattttgacatttatgatgaggatgaaaatcagagcccccgcagctttcaaaagaaaacacgacactattttattgctgcagtggagaggctctgggattatgggatgagtagctccccacatgttctaagaaacagggctcagagtggcagtgtccctcagttcaagaaagttgttttccaggaatttactgatggctcctttactcagcccttataccgtggagaactaaatgaacatttgggactcctggggccatatataagagcagaagttgaagataatatcatggtaactttcagaaatcaggcctctcgtccctattccttctattctagccttatttcttatgaggaagatcagaggcaaggagcagaacctagaaaaaactttgtcaagcctaatgaaaccaaaacttacttttggaaagtgcaacatcatatggcacccactaaagatgagtttgactgcaaagcctgggcttatttctctgatgttgacctggaaaaagatgtgcactcaggcctgattggaccccttctggtctgccacactaacacactgaaccctgctcatgggagacaagtgacagtacaggaatttgctctgtttttcaccatctttgatgagaccaaaagctggtacttcactgaaaatatggaaagaaactgcagggctccctgcaatatccagatggaagatcccacttttaaagagaattatcgcttccatgcaatcaatggctacataatggatacactacctggcttagtaatggctcaggatcaaaggattcgatggtatctgctcagcatgggcagcaatgaaaacatccattctattcatttcagtggacatgtgttcactgtacgaaaaaaagaggagtataaaatggcactgtacaatctctatccaggtgtttttgagacagtggaaatgttaccatccaaagctggaatttggcgggtggaatgccttattggcgagcatctacatgctgggatgagcacactttttctggtgtacagcaataagtgtcagactcccctgggaatggcttctggacacattagagattttcagattacagcttcaggacaatatggacagtgggccccaaagctggccagacttcattattccggatcaatcaatgcctggagcaccaaggagcccttttcttggatcaaggtggatctgttggcaccaatgattattcacggcatcaagacccagggtgcccgtcagaagttctccagcctctacatctctcagtttatcatcatgtatagtcttgatgggaagaagtggcagacttatcgaggaaattccactggaaccttaatggtcttctttggcaatgtggattcatctgggataaaacacaatatttttaaccctccaattattgctcgatacatccgtttgcacccaactcattatagcattcgcagcactcttcgcatggagttgatgggctgtgatttaaatagttgcagcatgccattgggaatggagagtaaagcaatatcagatgcacagattactgcttcatcctactttaccaatatgtttgccacctggtctccttcaaaagctcgacttcacctccaagggaggagtaatgcctggagacctcaggtgaataatccaaaagagtggctgcaagtggacttccagaagacaatgaaagtcacaggagtaactactcagggagtaaaatctctgcttaccagcatgtatgtgaaggagttcctcatctccagcagtcaagatggccatcagtggactctcttttttcagaatggcaaagtaaaggtttttcagggaaatcaagactccttcacacctgtggtgaactctctagacccaccgttactgactcgctaccttcgaattcacccccagagttgggtgcaccagattgccctgaggatggaggttctgggctgcgaggcacaggacctctactga

SEQ ID NO: 16 - DNA, 4375 bp, Artificial Sequence
  synthetic mcoHSQ
atgcagattgagctcagcacctgcttctttctgtgcctgctcaggttctgcttttcagccacaaggagatactatctgggagctgtggaactgtcatgggattacatgcagagtgacctgggagagctccctgtggatgctaggttccccccaagggtcccaaagtctttcccttttaataccagtgtggtctataagaaaacactctttgtggaatttactgatcacctgttcaacattgcaaagccaaggcctccctggatgggactgctgggacctaccatccaggctgaggtgtatgacactgtggtcatcacactgaaaaacatggcatctcaccctgtcagcctgcatgcagtgggagtcagctactggaaggcttcagaaggggcagagtatgatgatcagacaagccagagagaaaaagaggatgataaggtgttcccaggagggagccatacttatgtgtggcaggtcctgaaggagaatggcccaatggccagtgacccactgtgcctcacctactcatatctgagtcatgtggacctggtcaaggatctcaactcaggcctgattggggcactgctggtgtgcagggaaggctcactggccaaggagaaaacccagacactgcataagttcatcctgctctttgctgtgtttgatgaagggaaatcttggcacagtgagaccaagaacagtctgatgcaggacagggatgctgcttctgccagagcttggcccaagatgcacacagtgaatggatatgtcaataggtccctgccaggactcattggctgccacagaaagtcagtgtattggcatgtcattggaatgggcaccacaccagaagtgcacagcatcttcctggaggggcatacctttctggtcaggaaccacaggcaggccagcctggagatcagcccaatcaccttcctgacagcccagactctgctcatggatctggggcagttcctgctcttttgccacatcagctcccaccagcatgatggaatggaggcatatgtgaaagtggactcctgcccagaggaaccacagctgaggatgaagaacaatgaggaagctgaagactatgatgatgacctgacagactcagagatggatgtggtcaggtttgatgatgataacagcccctcctttatccagatcagaagtgtggccaagaaacacccaaagacatgggtccattacattgcagctgaggaagaggactgggattatgcacctctggtgctggccccagatgatagatcctacaaatcacagtatctgaacaatggaccccagaggattggcagaaagtacaagaaagtgaggttcatggcctatactgatgaaacatttaagactagagaagctatccagcatgagtcaggcatcctgggaccactgctctatggagaagtgggggacaccctgctcatcatcttcaagaaccaggcttccaggccatacaatatctatcctcatggcatcacagatgtgagaccactctactcaaggagactgcctaagggagtcaaacacctcaaggacttccctatcctgccaggggaaatctttaagtataaatggactgtgacagtggaggatgggcccactaagagtgacccaaggtgcctgaccagatactattcaagttttgtgaatatggaaagggatctggcatcaggactgattggacctctgctcatctgctacaaagagagtgtggatcagaggggcaaccagatcatgtcagacaagaggaatgtgatcctgttcagtgtctttgatgaaaacaggtcttggtatctgacagagaacatccagagattcctgccaaatcctgcaggggtgcagctggaagatccagagtttcaggcctcaaacatcatgcatagtatcaatggatatgtgtttgacagtctgcagctctctgtgtgcctgcatgaagtggcctactggtatatcctgtccattggagctcagacagatttcctgagtgtgttcttttcaggctacacttttaagcataaaatggtctatgaggacacactgactctcttcccttttagtggggaaacagtgtttatgagcatggagaatccagggctgtggattctgggatgccacaacagtgatttcaggaatagaggcatgactgctctgctcaaagtgtctagctgtgacaagaacacaggggactactatgaagattcttatgaggacatcagtgcttatctgctctccaaaaacaatgcaattgaacccagatcattcagtcagaatccacctgtgctgaagaggcaccagagagagatcactaggactaccctgcagtcagatcaggaagagattgactatgatgataccatctcagtggaaatgaagaaagaggactttgatatctatgatgaagatgagaaccagagtccaaggtctttccagaagaaaaccagacattactttattgctgcagtggagaggctgtgggattatggaatgtcctcaagtccacatgtgctgaggaatagggcacagtctggcagtgtccctcagttcaagaaagtggtcttccaggagtttacagatggcagcttcactcagcctctgtacaggggagaactcaatgagcacctggggctgctgggaccctatatcagagctgaagtggaggataacatcatggtcaccttcaggaatcaggcttcaagaccctacagtttttattctagcctgatcagctatgaagaggaccagaggcagggagctgaacctaggaaaaactttgtgaagccaaatgagaccaaaacatacttttggaaggtccagcaccacatggcaccaaccaaagatgagtttgattgcaaggcatgggcctatttttcagatgtggatctggagaaggatgtccacagtggcctcattgggcctctgctggtgtgccatactaacaccctgaatccagctcatggcaggcaggtgacagtccaggagtttgcactgttctttaccatctttgatgagacaaagtcctggtacttcactgaaaacatggagaggaattgcagagctccttgcaacatccagatggaagaccccaccttcaaggagaactacagatttcatgcaatcaatgggtatatcatggatacactgccaggactggtgatggcccaggaccagaggatcagatggtatctgctcagcatggggtccaatgagaatatccactctatccatttcagtggacatgtgtttacagtcagaaagaaagaagagtataaaatggccctgtacaacctctatccaggagtgtttgaaacagtggagatgctgccaagcaaggctgggatctggagggtggaatgcctcattggggagcacctgcatgcaggaatgtcaaccctgtttctggtctacagtaataagtgccagacacctctgggaatggcaagtggacatatcagggatttccagatcactgctagtggacagtatggacagtgggcaccaaagctggctagactccactattcaggctcaatcaatgcttggtccaccaaagagccattctcatggatcaaggtggacctgctggctcctatgatcatccatggcatcaaaacacagggggcaaggcagaagttctcctcactgtacatctctcagtttatcatcatgtatagcctggatggcaagaaatggcagacctacaggggcaatagcacagggactctgatggtgttctttggcaatgtggacagcagtgggatcaagcacaacatcttcaatcccccaatcattgcaaggtacatcagactgcaccccacccattattcaatcaggagtacactcaggatggaactgatggggtgtgatctcaacagttgctctatgccactgggaatggagtccaaggcaatctcagatgcccagatcactgctagctcctacttcactaatatgtttgctacctggagcccctccaaagcaaggctgcacctccagggaaggagcaatgcatggaggcctcaggtgaacaatcccaaggaatggctgcaggtggatttccagaaaactatgaaggtgactggagtcacaactcagggagtgaaaagtctgctcacttctatgtatgtcaaggagttcctgatctcaagttctcaggatggccaccagtggaccctgttctttcagaatggaaaggtgaaagtcttccagggcaatcaggattcctttacaccagtggtcaactcactggaccctcccctgctcactagatatctgagaatccaccctcagagctgggtgcatcagattgctctcagaatggaagtcctgggctgtgaggcacaggacctgtattgag

SEQ ID NO: 17 - DNA, 2903 bp, Artificial Sequence
  synthetic 6x-tRNA
gtcgactacgtagaatccggagccgtctttgtcttccagctccatcttttccaccttttgcttaggcagtcccccgagtcgtgtcaaggctgaggagtagaaatggaacagcactaatattaatggcaaaaccgttgtgaaatagggttactttctgtttaagcaaggaaaataaagtaaagcaatgggaaaaaaattaaaagcaaaaggaatggaggtgccggggattgaacccggggcctcgtgcatgctaagcacgcgctctaccactgagctacacccccgtactgaaacggttctctcgagagtatattcaagatcagaatctgacccttttgctaggtttcagaaccattagttgtaatcagccaaggtctattttatttagttatttctgatatctcaaatttaggttttgcgtccctctttgctgacagctgagcaaaccgcattctacaccgaaggccctctattgatggccctgatttaaatcccttccgccgcctgccgcaggtggctagggtctgagcacacttgaacctcacacccgccccaggggtagctccttggttcccttcagccccgatgtgtccctcgtgctttgaaatggaattacagttttggttaaaaacatgccttttccgagttaggaagaatctaaatcgactgaacgccagtctaaaatttcggcgttcccacaccgggagtcgaacccgggccgcctgggtgaaaaccaggaatcctaaccgctagaccatgtgggagacggcaatagcgactccaagcctagacaaattgagtcttctcggtcggcttccgcccactccatcgcgttcatccgtaggcgtcaaacctgctcctgcgcctgcgcggagtctgcagcggtttaaaccgttcaggttcgcattctactgtttctctccttgcaggggcccttgaatctttcttcaatctactctcgcgtgcccgggcgactgggcataaccctacaggttcatgtggggtgggtggcgcgcgctagcggtgaaggtcactcacaattgcgcgctgggcagacgacggcagccattacttttacctcgatcgctgttttcctggatccgcacgggtccaacccgactcatcccaaccaacctgaggtatgaaaaccaggaaagagagctagcaccggagcgttggtggtatagtggtaagcatagctgccttccaagcagttgacccgggttcgattcccggccaacgcaagtcgttttgggtgttttttcccccccccgccttttccttttcgtgttttctgggccccagcatcgttgagggttttcgtgaggttttcctgaggaaacttccgctccgaaaggacccactttccgctacacccgcgaccacggctggaccaccgcgctcctgacggatgcgccctgcaagcccctccaggcgagagcaggccggcctgtgctcagttttgtagcatcaaaactaggatttctcttgttacccccagtcactccattcagttttcgtgtctttcccagctgcatccatcctttcctcattttcgtatgcagccgactttttgtgacatctttgtattcattctctgcaattcagctgacctggccaaggaaacaagatcctaagcgtctttccggcggcgccgtggcttagttggttaaagcgcctgtctagtaaacaggagatcctgggttcgaatcccagcggtgcctccgtgtttcccccacgcttttgccaacattaaacattgtgaggacagttgcagaaactcataacttccatcctacatggtttactcacgtacccatctatcctctcccggtgcatctgccacacgctgttgggtttttgctcttcgtgcacatggtacttgcgcctcgacctgcagttacaccagtcgcatcatctgtacagcgctaaaacctagctgggcgtggtggtcctgcagtcccagctactcgggaggctgaggcaggagaatggcttgaatccaggaggcggaggtggcagtgagccgagattgcgccactgcactccagcctggtgacagagcgagactccatctcaaaaaaaaaaaaaaaaaaaaagtcagaattaggtactaaaagccatatgacatgcctgaacagggacttgaaccctggaccctcagattaaaagtctgatgctctaccaactgagctatccaggcttcttccctgctagtttattttaatgcagtaataaataacagcactttgttaaaaataataaaggtataatctgtgacacatccaaagtggacaagatgaagagataataggtatacaccaggattcccctgggcaaactgggacctcttggtaccctatatattaagagtctcgggttttgttttcacttaagcaaatggttaacgaattagcaggttaagaaaaactgtttccccgtaagaagcagggttctttggtgttcaatgtggagctccgccactcccagcccgggtgaaggaaaactgggaaacagaatgaatgtgattatctattcgaagataaatttccacaaagcatgccgtttgatagtagcttataatgtggaagtaaggcatcctgtcatccggccggttagctcagttggttagagcgtggtgctaataacgccaaggtcgcgggttcgatccccgtactggccaagtattctctgtggcttttatcaccagaatggatagtaacccagacatcgatctaaacgtgtacctgtgtgtttctccaggcttaactttgccccgagaaaacggatctgtgaatttggtgcgccctcgcttactcgacagcggttaatttgaacggggacgtttctttccgctgcctccaaggcatacccacatcctaccacgatggtggcggccgcaa

SEQ ID NO: 18 - protein, 1467 aa, Artificial Sequence
  synthetic HP44/OL aa
MQLELSTCVFLCLLPLGFSAIRRYYLGAVELSWDYRQSELLRELHVDTRFPATAPGALPLGPSVLYKKTVFVEFTDQLFSVARPRPPWMGLLGPTIQAEVYDTVVVTLKNMASHPVSLHAVGVSFWKSSEGAEYEDHTSQREKEDDKVLPGKSQTYVWQVLKENGPTASDPPCLTYSYLSHVDLVKDLNSGLIGALLVCREGSLTRERTQNLHEFVLLFAVFDEGKSWHSARNDSWTRAMDPAPARAQPAMHTVNGYVNRSLPGLIGCHKKSVYWHVIGMGTSPEVHSIFLEGHTFLVRHHRQASLEISPLTFLTAQTFLMDLGQFLLFCHISSHHHGGMEAHVRVESCAEEPQLRRKADEEEDYDDNLYDSDMDVVRLDGDDVSPFIQIRSVAKKHPKTWVHYISAEEEDWDYAPAVPSPSDRSYKSLYLNSGPQRIGRKYKKARFVAYTDVTFKTRKAIPYESGILGPLLYGEVGDTLLIIFKNKASRPYNIYPHGITDVSALHPGRLLKGWKHLKDMPILPGETFKYKWTVTVEDGPTKSDPRCLTRYYSSSINLEKDLASGLIGPLLICYKESVDQRGNQMMSDKRNVILFSVFDENQSWYLAENIQRFLPNPDGLQPQDPEFQASNIMHSINGYVFDSLQLSVCLHEVAYWYILSVGAQTDFLSVFFSGYTFKHKMVYEDTLTLFPFSGETVFMSMENPGLWVLGCHNSDLRNRGMTALLKVYSCDRDIGDYYDNTYEDIPGFLLSGKNVIEPRSFAQNSRPPSASAPKPPVLRRHQRDISLPTFQPEEDKMDYDDIFSTETKGEDFDIYGEDENQDPRSFQKRTRHYFIAAVEQLWDYGMSESPRALRNRAQNGEVPRFKKVVFREFADGSFTQPSYRGELNKHLGLLGPYIRAEVEDNIMVTFKNQASRPYSFYSSLISYPDDQEQGAEPRHNFVQPNETRTYFWKVQHHMAPTEDEFDCKAWAYFSDVDLEKDVHSGLIGPLLICRANTLNAAHGRQVTVQEFALFFTIFDETKSWYFTENVERNCRAPCHLQMEDPTLKENYRFHAINGYVMDTLPGLVMAQNQRIRWYLLSMGSNENIHSIHFSGHVFSVRKKEEYKMAVYNLYPGVFETVEMLPSKVGIWRIECLIGEHLQAGMSTTFLVYSKKCQTPLGMASGHIRDFQITASGQYGQWAPKLARLHYSGSINAWSTKEPFSWIKVDLLAPMIIHGIKTQGARQKFSSLYISQFIIMYSLDGKKWQTYRGNSTGTLMVFFGNVDSSGIKHNIFNPPIIARYIRLHPTHYSIRSTLRMELMGCDLNSCSMPLGMESKAISDAQITASSYFTNMFATWSPSKARLHLQGRSNAWRPQVNNPKEWLQVDFQKTMKVTGVTTQGVKSLLTSMYVKEFLISSSQDGHQWTLFFQNGKVKVFQGNQDSFTPVVNSLDPPLLTRYLRIHPQSWVHQIALRMEVLGCEAQDLY

SEQ ID NO: 19 - DNA, 4401 bp, Artificial Sequence
  synthetic HP44/OL NT
atgcagctagagctctccacctgtgtctttctgtgtctcttgccactcggctttagtgccatcaggagatactacctgggcgcagtggaactgtcctgggactaccggcaaagtgaactcctccgtgagctgcacgtggacaccagatttcctgctacagcgccaggagctcttccgttgggcccgtcagtcctgtacaaaaagactgtgttcgtagagttcacggatcaacttttcagcgttgccaggcccaggccaccatggatgggtctgctgggtcctaccatccaggctgaggtttacgacacggtggtcgttaccctgaagaacatggcttctcatcccgttagtcttcacgctgtcggcgtctccttctggaaatcttccgaaggcgctgaatatgaggatcacaccagccaaagggagaaggaagacgataaagtccttcccggtaaaagccaaacctacgtctggcaggtcctgaaagaaaatggtccaacagcctctgacccaccatgtcttacctactcatacctgtctcacgtggacctggtgaaagacctgaattcgggcctcattggagccctgctggtttgtagagaagggagtctgaccagagaaaggacccagaacctgcacgaatttgtactactttttgctgtctttgatgaagggaaaagttggcactcagcaagaaatgactcctggacacgggccatggatcccgcacctgccagggcccagcctgcaatgcacacagtcaatggctatgtcaacaggtctctgccaggtctgatcggatgtcataagaaatcagtctactggcacgtgattggaatgggcaccagcccggaagtgcactccatttttcttgaaggccacacgtttctcgtgaggcaccatcgccaggcttccttggagatctcgccactaactttcctcactgctcagacattcctgatggaccttggccagttcctactgttttgtcatatctcttcccaccaccatggtggcatggaggctcacgtcagagtagaaagctgcgccgaggagccccagctgcggaggaaagctgatgaagaggaagattatgatgacaatttgtacgactcggacatggacgtggtccggctcgatggtgacgacgtgtctccctttatccaaatccgctcggttgccaagaagcatcccaaaacctgggtgcactacatctctgcagaggaggaggactgggactacgcccccgcggtccccagccccagtgacagaagttataaaagtctctacttgaacagtggtcctcagcgaattggtaggaaatacaaaaaagctcgattcgtcgcttacacggatgtaacatttaagactcgtaaagctattccgtatgaatcaggaatcctgggacctttactttatggagaagttggagacacacttttgattatatttaagaataaagcgagccgaccatataacatctaccctcatggaatcactgatgtcagcgctttgcacccagggagacttctaaaaggttggaaacatttgaaagacatgccaattctgccaggagagactttcaagtataaatggacagtgactgtggaagatgggccaaccaagtccgatcctcggtgcctgacccgctactactcgagctccattaatctagagaaagatctggcttcgggactcattggccctctcctcatctgctacaaagaatctgtagaccaaagaggaaaccagatgatgtcagacaagagaaacgtcatcctgttttctgtattcgatgagaatcaaagctggtacctcgcagagaatattcagcgcttcctccccaatccggatggattacagccccaggatccagagttccaagcttctaacatcatgcacagcatcaatggctatgtttttgatagcttgcagctgtcggtttgtttgcacgaggtggcatactggtacattctaagtgttggagcacagacggacttcctctccgtcttcttctctggctacaccttcaaacacaaaatggtctatgaagacacactcaccctgttccccttctcaggagaaacggtcttcatgtcaatggaaaacccaggtctctgggtccttgggtgccacaactcagacttgcggaacagagggatgacagccttactgaaggtgtatagttgtgacagggacattggtgattattatgacaacacttatgaagatattccaggcttcttgctgagtggaaagaatgtcattgaacctaggagctttgcccagaattcaagaccccctagtgcgagcgctccaaagcctccggtcctgcgacggcatcagagggacataagccttcctacttttcagccggaggaagacaaaatggactatgatgatatcttctcaactgaaacgaagggagaagattttgacatttacggtgaggatgaaaatcaggaccctcgcagctttcagaagagaacccgacactatttcattgctgcggtggagcagctctgggattacgggatgagcgaatccccccgggcgctaagaaacagggctcagaacggagaggtgcctcggttcaagaaggtggtcttccgggaatttgctgacggctccttcacgcagccgtcgtaccgcggggaactcaacaaacacttggggctcttgggaccctacatcagagcggaagttgaagacaacatcatggtaactttcaaaaaccaggcgtctcgtccctattccttctactcgagccttatttcttatccggatgatcaggagcaaggggcagaacctcgacacaacttcgtccagccaaatgaaaccagaacttacttttggaaagtgcagcatcacatggcacccacagaagacgagtttgactgcaaagcctgggcctacttttctgatgttgacctggaaaaagatgtgcactcaggcttgatcggcccccttctgatctgccgcgccaacaccctgaacgctgctcacggtagacaagtgaccgtgcaagaatttgctctgtttttcactatttttgatgagacaaagagctggtacttcactgaaaatgtggaaaggaactgccgggccccctgccatctgcagatggaggaccccactctgaaagaaaactatcgcttccatgcaatcaatggctatgtgatggatacactccctggcttagtaatggctcagaatcaaaggatccgatggtatctgctcagcatgggcagcaatgaaaatatccattcgattcattttagcggacacgtgttcagtgtacggaaaaaggaggagtataaaatggccgtgtacaatctctatccgggtgtctttgagacagtggaaatgctaccgtccaaagttggaatttggcgaatagaatgcctgattggcgagcacctgcaagctgggatgagcacgactttcctggtgtacagcaagaagtgtcagactcccctgggaatggcttctggacacattagagattttcagattacagcttcaggacaatatggacagtgggccccaaagctggccagacttcattattccggatcaatcaatgcctggagcaccaaggagcccttttcttggatcaaggtggatctgttggcaccaatgattattcacggcatcaagacccagggtgcccgtcagaagttctccagcctctacatctctcagtttatcatcatgtatagtcttgatgggaagaagtggcagacttatcgaggaaattccactggaaccttaatggtcttctttggcaatgtggattcatctgggataaaacacaatatttttaaccctccaattattgctcgatacatccgtttgcacccaactcattatagcattcgcagcactcttcgcatggagttgatgggctgtgatttaaatagttgcagcatgccattgggaatggagagtaaagcaatatcagatgcacagattactgcttcatcctactttaccaatatgtttgccacctggtctccttcaaaagctcgacttcacctccaagggaggagtaatgcctggagacctcaggtgaataatccaaaagagtggctgcaagtggacttccagaagacaatgaaagtcacaggagtaactactcagggagtaaaatctctgcttaccagcatgtatgtgaaggagttcctcatctccagcagtcaagatggccatcagtggactctcttttttcagaatggcaaagtaaaggtttttcagggaaatcaagactccttcacacctgtggtgaactctctagacccaccgttactgactcgctaccttcgaattcacccccagagttgggtgcaccagattgccctgaggatggaggttctgggctgcgaggcacaggacctctac

SEQ ID NO: 20 - protein, 1457 aa, Artificial Sequence
  synthetic HP46/SQ aa
MQLELSTCVFLCLLPLGFSAIRRYYLGAVELSWDYRQSELLRELHVDTRFPATAPGALPLGPSVLYKKTVFVEFTDQLFSVARPRPPWMGLLGPTIQAEVYDTVVVTLKNMASHPVSLHAVGVSFWKSSEGAEYEDHTSQREKEDDKVLPGKSQTYVWQVLKENGPTASDPPCLTYSYLSHVDLVKDLNSGLIGALLVCREGSLTRERTQNLHEFVLLFAVFDEGKSWHSARNDSWTRAMDPAPARAQPAMHTVNGYVNRSLPGLIGCHKKSVYWHVIGMGTSPEVHSIFLEGHTFLVRHHRQASLEISPLTFLTAQTFLMDLGQFLLFCHISSHHHGGMEAHVRVESCAEEPQLRRKADEEEDYDDNLYDSDMDVVRLDGDDVSPFIQIRSVAKKHPKTWVHYIAAEEEDWDYAPLVLAPDDRSYKSQYLNNGPQRIGRKYKKVRFMAYTDETFKTREAIQHESGILGPLLYGEVGDTLLIIFKNQASRPYNIYPHGITDVRPLYSRRLPKGVKHLKDFPILPGEIFKYKWTVTVEDGPTKSDPRCLTRYYSSFVNMERDLASGLIGPLLICYKESVDQRGNQIMSDKRNVILFSVFDENRSWYLTENIQRFLPNPAGVQLEDPEFQASNIMHSINGYVFDSLQLSVCLHEVAYWYILSIGAQTDFLSVFFSGYTFKHKMVYEDTLTLFPFSGETVFMSMENPGLWILGCHNSDFRNRGMTALLKVSSCDKNTGDYYEDSYEDISAYLLSKNNAIEPRSFSQNPPVLKRHQREITRTTLQSDQEEIDYDDTISVEMKKEDFDIYDEDENQSPRSFQKKTRHYFIAAVERLWDYGMSSSPHVLRNRAQSGSVPQFKKVVFQEFTDGSFTQPLYRGELNEHLGLLGPYIRAEVEDNIMVTFRNQASRPYSFYSSLISYEEDQRQGAEPRKNFVKPNETKTYFWKVQHHMAPTKDEFDCKAWAYFSDVDLEKDVHSGLIGPLLVCHTNTLNPAHGRQVTVQEFALFFTIFDETKSWYFTENMERNCRAPCNIQMEDPTFKENYRFHAINGYIMDTLPGLVMAQDQRIRWYLLSMGSNENIHSIHFSGHVFTVRKKEEYKMALYNLYPGVFETVEMLPSKAGIWRVECLIGEHLHAGMSTLFLVYSNKCQTPLGMASGHIRDFQITASGQYGQWAPKLARLHYSGSINAWSTKEPFSWIKVDLLAPMIIHGIKTQGARQKFSSLYISQFIIMYSLDGKKWQTYRGNSTGTLMVFFGNVDSSGIKHNIFNPPIIARYIRLHPTHYSIRSTLRMELMGCDLNSCSMPLGMESKAISDAQITASSYFTNMFATWSPSKARLHLQGRSNAWRPQVNNPKEWLQVDFQKTMKVTGVTTQGVKSLLTSMYVKEFLISSSQDGHQWTLFFQNGKVKVFQGNQDSFTPVVNSLDPPLLTRYLRIHPQSWVHQIALRMEVLGCEAQDLY

SEQ ID NO: 21 - DNA, 4368 bp, Artificial Sequence
  synthetic HP46/SQ NT
atgcagctagagctctccacctgtgtctttctgtgtctcttgccactcggctttagtgccatcaggagatactacctgggcgcagtggaactgtcctgggactaccggcaaagtgaactcctccgtgagctgcacgtggacaccagatttcctgctacagcgccaggagctcttccgttgggcccgtcagtcctgtacaaaaagactgtgttcgtagagttcacggatcaacttttcagcgttgccaggcccaggccaccatggatgggtctgctgggtcctaccatccaggctgaggtttacgacacggtggtcgttaccctgaagaacatggcttctcatcccgttagtcttcacgctgtcggcgtctccttctggaaatcttccgaaggcgctgaatatgaggatcacaccagccaaagggagaaggaagacgataaagtccttcccggtaaaagccaaacctacgtctggcaggtcctgaaagaaaatggtccaacagcctctgacccaccatgtcttacctactcatacctgtctcacgtggacctggtgaaagacctgaattcgggcctcattggagccctgctggtttgtagagaagggagtctgaccagagaaaggacccagaacctgcacgaatttgtactactttttgctgtctttgatgaagggaaaagttggcactcagcaagaaatgactcctggacacgggccatggatcccgcacctgccagggcccagcctgcaatgcacacagtcaatggctatgtcaacaggtctctgccaggtctgatcggatgtcataagaaatcagtctactggcacgtgattggaatgggcaccagcccggaagtgcactccatttttcttgaaggccacacgtttctcgtgaggcaccatcgccaggcttccttggagatctcgccactaactttcctcactgctcagacattcctgatggaccttggccagttcctactgttttgtcatatctcttcccaccaccatggtggcatggaggctcacgtcagagtagaaagctgcgccgaggagccccagctgcggaggaaagctgatgaagaggaagattatgatgacaatttgtacgactcggacatggacgtggtccggctcgatggtgacgacgtgtctccctttatccaaatccgctcagttgccaagaagcatcctaaaacttgggtacattacattgctgctgaagaggaggactgggactatgctcccttagtcctcgcccccgatgacagaagttataaaagtcaatatttgaacaatggccctcagcggattggtaggaagtacaaaaaagtccgatttatggcatacacagatgaaacctttaagacgcgtgaagctattcagcatgaatcaggaatcttgggacctttactttatggggaagttggagacacactgttgattatatttaagaatcaagcaagcagaccatataacatctaccctcacggaatcactgatgtccgtcctttgtattcaaggagattaccaaaaggtgtaaaacatttgaaggattttccaattctgccaggagaaatattcaaatataaatggacagtgactgtagaagatgggccaactaaatcagatccgcggtgcctgacccgctattactctagtttcgttaatatggagagagatctagcttcaggactcattggccctctcctcatctgctacaaagaatctgtagatcaaagaggaaaccagataatgtcagacaagaggaatgtcatcctgttttctgtatttgatgagaaccgaagctggtacctcacagagaatatacaacgctttctccccaatccagctggagtgcagcttgaggatccagagttccaagcctccaacatcatgcacagcatcaatggctatgtttttgatagtttgcagttgtcagtttgtttgcatgaggtggcatactggtacattctaagcattggagcacagactgacttcctttctgtcttcttctctggatataccttcaaacacaaaatggtctatgaagacacactcaccctattcccattctcaggagaaactgtcttcatgtcgatggaaaacccaggtctatggattctggggtgccacaactcagactttcggaacagaggcatgaccgccttactgaaggtttctagttgtgacaagaacactggtgattattacgaggacagttatgaagatatttcagcatacttgctgagtaaaaacaatgccattgaacctaggagcttctctcagaatccaccagtcttgaaacgccatcaacgggaaataactcgtactactcttcagtcagatcaagaggaaattgactatgatgataccatatcagttgaaatgaagaaggaagattttgacatttatgatgaggatgaaaatcagagcccccgcagctttcaaaagaaaacacgacactattttattgctgcagtggagaggctctgggattatgggatgagtagctccccacatgttctaagaaacagggctcagagtggcagtgtccctcagttcaagaaagttgttttccaggaatttactgatggctcctttactcagcccttataccgtggagaactaaatgaacatttgggactcctggggccatatataagagcagaagttgaagataatatcatggtaactttcagaaatcaggcctctcgtccctattccttctattctagccttatttcttatgaggaagatcagaggcaaggagcagaacctagaaaaaactttgtcaagcctaatgaaaccaaaacttacttttggaaagtgcaacatcatatggcacccactaaagatgagtttgactgcaaagcctgggcttatttctctgatgttgacctggaaaaagatgtgcactcaggcctgattggaccccttctggtctgccacactaacacactgaaccctgctcatgggagacaagtgacagtacaggaatttgctctgtttttcaccatctttgatgagaccaaaagctggtacttcactgaaaatatggaaagaaactgcagggctccctgcaatatccagatggaagatcccacttttaaagagaattatcgcttccatgcaatcaatggctacataatggatacactacctggcttagtaatggctcaggatcaaaggattcgatggtatctgctcagcatgggcagcaatgaaaacatccattctattcatttcagtggacatgtgttcactgtacgaaaaaaagaggagtataaaatggcactgtacaatctctatccaggtgtttttgagacagtggaaatgttaccatccaaagctggaatttggcgggtggaatgccttattggcgagcatctacatgctgggatgagcacactttttctggtgtacagcaataagtgtcagactcccctgggaatggcttctggacacattagagattttcagattacagcttcaggacaatatggacagtgggccccaaagctggccagacttcattattccggatcaatcaatgcctggagcaccaaggagcccttttcttggatcaaggtggatctgttggcaccaatgattattcacggcatcaagacccagggtgcccgtcagaagttctccagcctctacatctctcagtttatcatcatgtatagtcttgatgggaagaagtggcagacttatcgaggaaattccactggaaccttaatggtcttctttggcaatgtggattcatctgggataaaacacaatatttttaaccctccaattattgctcgatacatccgtttgcacccaactcattatagcattcgcagcactcttcgcatggagttgatgggctgtgatttaaatagttgcagcatgccattgggaatggagagtaaagcaatatcagatgcacagattactgcttcatcctactttaccaatatgtttgccacctggtctccttcaaaagctcgacttcacctccaagggaggagtaatgcctggagacctcaggtgaataatccaaaagagtggctgcaagtggacttccagaagacaatgaaagtcacaggagtaactactcagggagtaaaatctctgcttaccagcatgtatgtgaaggagttcctcatctccagcagtcaagatggccatcagtggactctcttttttcagaatggcaaagtaaaggtttttcagggaaatcaagactccttcacacctgtggtgaactctctagacccaccgttactgactcgctaccttcgaattcacccccagagttgggtgcaccagattgccctgaggatggaggttctgggctgcgaggcacaggacctc

SEQ ID NO: 22 - protein, 1467 aa, Artificial Sequence
  synthetic HP47/OL aa
MQLELSTCVFLCLLPLGFSAIRRYYLGAVELSWDYRQSELLRELHVDTRFPATAPGALPLGPSVLYKKTVFVEFTDQLFSVARPRPPWMGLLGPTIQAEVYDTVVVTLKNMASHPVSLHAVGVSFWKSSEGAEYEDHTSQREKEDDKVLPGKSQTYVWQVLKENGPTASDPPCLTYSYLSHVDLVKDLNSGLIGALLVCREGSLTRERTQNLHEFVLLFAVFDEGKSWHSARNDSWTRAMDPAPARAQPAMHTVNGYVNRSLPGLIGCHKKSVYWHVIGMGTSPEVHSIFLEGHTFLVRHHRQASLEISPLTFLTAQTFLMDLGQFLLFCHISSHHHGGMEAHVRVESCAEEPQLRRKADEEEDYDDNLYDSDMDVVRLDGDDVSPFIQIRSVAKKHPKTWVHYIAAEEEDWDYAPLVLAPDDRSYKSQYLNNGPQRIGRKYKKVRFMAYTDETFKTREAIQHESGILGPLLYGEVGDTLLIIFKNQASRPYNIYPHGITDVRPLYSRRLPKGVKHLKDFPILPGEIFKYKWTVTVEDGPTKSDPRCLTRYYSSFVNMERDLASGLIGPLLICYKESVDQRGNQIMSDKRNVILFSVFDENRSWYLTENIQRFLPNPAGVQLEDPEFQASNIMHSINGYVFDSLQLSVCLHEVAYWYILSIGAQTDFLSVFFSGYTFKHKMVYEDTLTLFPFSGETVFMSMENPGLWILGCHNSDFRNRGMTALLKVSSCDKNTGDYYEDSYEDISAYLLSKNNAIEPRSFAQNSRPPSASAPKPPVLRRHQRDISLPTFQPEEDKMDYDDIFSTETKGEDFDIYGEDENQDPRSFQKRTRHYFIAAVEQLWDYGMSESPRALRNRAQNGEVPRFKKVVFREFADGSFTQPSYRGELNKHLGLLGPYIRAEVEDNIMVTFKNQASRPYSFYSSLISYPDDQEQGAEPRHNFVQPNETRTYFWKVQHHMAPTEDEFDCKAWAYFSDVDLEKDVHSGLIGPLLICRANTLNAAHGRQVTVQEFALFFTIFDETKSWYFTENVERNCRAPCHLQMEDPTLKENYRFHAINGYVMDTLPGLVMAQNQRIRWYLLSMGSNENIHSIHFSGHVFSVRKKEEYKMAVYNLYPGVFETVEMLPSKVGIWRIECLIGEHLQAGMSTTFLVYSKKCQTPLGMASGHIRDFQITASGQYGQWAPKLARLHYSGSINAWSTKEPFSWIKVDLLAPMIIHGIKTQGARQKFSSLYISQFIIMYSLDGKKWQTYRGNSTGTLMVFFGNVDSSGIKHNIFNPPIIARYIRLHPTHYSIRSTLRMELMGCDLNSCSMPLGMESKAISDAQITASSYFTNMFATWSPSKARLHLQGRSNAWRPQVNNPKEWLQVDFQKTMKVTGVTTQGVKSLLTSMYVKEFLISSSQDGHQWTLFFQNGKVKVFQGNQDSFTPVVNSLDPPLLTRYLRIHPQSWVHQIALRMEVLGCEAQDLY

SEQ ID NO: 23 - DNA, 4401 bp, Artificial Sequence
  synthetic HP47/OL NT
atgcagctagagctctccacctgtgtctttctgtgtctcttgccactcggctttagtgccatcaggagatactacctgggcgcagtggaactgtcctgggactaccggcaaagtgaactcctccgtgagctgcacgtggacaccagatttcctgctacagcgccaggagctcttccgttgggcccgtcagtcctgtacaaaaagactgtgttcgtagagttcacggatcaacttttcagcgttgccaggcccaggccaccatggatgggtctgctgggtcctaccatccaggctgaggtttacgacacggtggtcgttaccctgaagaacatggcttctcatcccgttagtcttcacgctgtcggcgtctccttctggaaatcttccgaaggcgctgaatatgaggatcacaccagccaaagggagaaggaagacgataaagtccttcccggtaaaagccaaacctacgtctggcaggtcctgaaagaaaatggtccaacagcctctgacccaccatgtcttacctactcatacctgtctcacgtggacctggtgaaagacctgaattcgggcctcattggagccctgctggtttgtagagaagggagtctgaccagagaaaggacccagaacctgcacgaatttgtactactttttgctgtctttgatgaagggaaaagttggcactcagcaagaaatgactcctggacacgggccatggatcccgcacctgccagggcccagcctgcaatgcacacagtcaatggctatgtcaacaggtctctgccaggtctgatcggatgtcataagaaatcagtctactggcacgtgattggaatgggcaccagcccggaagtgcactccatttttcttgaaggccacacgtttctcgtgaggcaccatcgccaggcttccttggagatctcgccactaactttcctcactgctcagacattcctgatggaccttggccagttcctactgttttgtcatatctcttcccaccaccatggtggcatggaggctcacgtcagagtagaaagctgcgccgaggagccccagctgcggaggaaagctgatgaagaggaagattatgatgacaatttgtacgactcggacatggacgtggtccggctcgatggtgacgacgtgtctccctttatccaaatccgctcagttgccaagaagcatcctaaaacttgggtacattacattgctgctgaagaggaggactgggactatgctcccttagtcctcgcccccgatgacagaagttataaaagtcaatatttgaacaatggccctcagcggattggtaggaagtacaaaaaagtccgatttatggcatacacagatgaaacctttaagacgcgtgaagctattcagcatgaatcaggaatcttgggacctttactttatggggaagttggagacacactgttgattatatttaagaatcaagcaagcagaccatataacatctaccctcacggaatcactgatgtccgtcctttgtattcaaggagattaccaaaaggtgtaaaacatttgaaggattttccaattctgccaggagaaatattcaaatataaatggacagtgactgtagaagatgggccaactaaatcagatccgcggtgcctgacccgctattactctagtttcgttaatatggagagagatctagcttcaggactcattggccctctcctcatctgctacaaagaatctgtagatcaaagaggaaaccagataatgtcagacaagaggaatgtcatcctgttttctgtatttgatgagaaccgaagctggtacctcacagagaatatacaacgctttctccccaatccagctggagtgcagcttgaggatccagagttccaagcctccaacatcatgcacagcatcaatggctatgtttttgatagtttgcagttgtcagtttgtttgcatgaggtggcatactggtacattctaagcattggagcacagactgacttcctttctgtcttcttctctggatataccttcaaacacaaaatggtctatgaagacacactcaccctattcccattctcaggagaaactgtcttcatgtcgatggaaaacccaggtctatggattctggggtgccacaactcagactttcggaacagaggcatgaccgccttactgaaggtttctagttgtgacaagaacactggtgattattacgaggacagttatgaagatatttcagcatacttgctgagtaaaaacaatgccattgaacctaggagctttgcccagaattcaagaccccctagtgcgagcgctccaaagcctccggtcctgcgacggcatcagagggacataagccttcctacttttcagccggaggaagacaaaatggactatgatgatatcttctcaactgaaacgaagggagaagattttgacatttacggtgaggatgaaaatcaggaccctcgcagctttcagaagagaacccgacactatttcattgctgcggtggagcagctctgggattacgggatgagcgaatccccccgggcgctaagaaacagggctcagaacggagaggtgcctcggttcaagaaggtggtcttccgggaatttgctgacggctccttcacgcagccgtcgtaccgcggggaactcaacaaacacttggggctcttgggaccctacatcagagcggaagttgaagacaacatcatggtaactttcaaaaaccaggcgtctcgtccctattccttctactcgagccttatttcttatccggatgatcaggagcaaggggcagaacctcgacacaacttcgtccagccaaatgaaaccagaacttacttttggaaagtgcagcatcacatggcacccacagaagacgagtttgactgcaaagcctgggcctacttttctgatgttgacctggaaaaagatgtgcactcaggcttgatcggcccccttctgatctgccgcgccaacaccctgaacgctgctcacggtagacaagtgaccgtgcaagaatttgctctgtttttcactatttttgatgagacaaagagctggtacttcactgaaaatgtggaaaggaactgccgggccccctgccatctgcagatggaggaccccactctgaaagaaaactatcgcttccatgcaatcaatggctatgtgatggatacactccctggcttagtaatggctcagaatcaaaggatccgatggtatctgctcagcatgggcagcaatgaaaatatccattcgattcattttagcggacacgtgttcagtgtacggaaaaaggaggagtataaaatggccgtgtacaatctctatccgggtgtctttgagacagtggaaatgctaccgtccaaagttggaatttggcgaatagaatgcctgattggcgagcacctgcaagctgggatgagcacgactttcctggtgtacagcaagaagtgtcagactcccctgggaatggcttctggacacattagagattttcagattacagcttcaggacaatatggacagtgggccccaaagctggccagacttcattattccggatcaatcaatgcctggagcaccaaggagcccttttcttggatcaaggtggatctgttggcaccaatgattattcacggcatcaagacccagggtgcccgtcagaagttctccagcctctacatctctcagtttatcatcatgtatagtcttgatgggaagaagtggcagacttatcgaggaaattccactggaaccttaatggtcttctttggcaatgtggattcatctgggataaaacacaatatttttaaccctccaattattgctcgatacatccgtttgcacccaactcattatagcattcgcagcactcttcgcatggagttgatgggctgtgatttaaatagttgcagcatgccattgggaatggagagtaaagcaatatcagatgcacagattactgcttcatcctactttaccaatatgtttgccacctggtctccttcaaaagctcgacttcacctccaagggaggagtaatgcctggagacctcaggtgaataatccaaaagagtggctgcaagtggacttccagaagacaatgaaagtcacaggagtaactactcagggagtaaaatctctgcttaccagcatgtatgtgaaggagttcctcatctccagcagtcaagatggccatcagtggactctcttttttcagaatggcaaagtaaaggtttttcagggaaatcaagactccttcacacctgtggtgaactctctagacccaccgttactgactcgctaccttcgaattcacccccagagttgggtgcaccagattgccctgaggatggaggttctgggctgcgaggcacaggacctctac

SEQ ID NO: 24 - protein, 1457 aa, Homo sapiens
MQIELSTCFFLCLLRFCFSATRRYYLGAVELSWDYMQSDLGELPVDARFPPRVPKSFPFNTSVVYKKTLFVEFTVHLFNIAKPRPPWMGLLGPTIQAEVYDTVVITLKNMASHPVSLHAVGVSYWKASEGAEYDDQTSQREKEDDKVFPGGSHTYVWQVLKENGPMASDPLCLTYSYLSHVDLVKDLNSGLIGALLVCREGSLAKEKTQTLHKFILLFAVFDEGKSWHSETKNSLMQDRDAASARAWPKMHTVNGYVNRSLPGLIGCHRKSVYWHVIGMGTTPEVHSIFLEGHTFLVRNHRQASLEISPITFLTAQTLLMDLGQFLLFCHISSHQHDGMEAYVKVDSCPEEPQLRMKNNEEAEDYDDDLTDSEMDVVRFDDDNSPSFIQIRSVAKKHPKTWVHYIAAEEEDWDYAPLVLAPDDRSYKSQYLNNGPQRIGRKYKKVRFMAYTDETFKTREAIQHESGILGPLLYGEVGDTLLIIFKNQASRPYNIYPHGITDVRPLYSRRLPKGVKHLKDFPILPGEIFKYKWTVTVEDGPTKSDPRCLTRYYSSFVNMERDLASGLIGPLLICYKESVDQRGNQIMSDKRNVILFSVFDENRSWYLTENIQRFLPNPAGVQLEDPEFQASNIMHSINGYVFDSLQLSVCLHEVAYWYILSIGAQTDFLSVFFSGYTFKHKMVYEDTLTLFPFSGETVFMSMENPGLWILGCHNSDFRNRGMTALLKVSSCDKNTGDYYEDSYEDISAYLLSKNNAIEPRSFSQNPPVLKRHQREITRTTLQSDQEEIDYDDTISVEMKKEDFDIYDEDENQSPRSFQKKTRHYFIAAVERLWDYGMSSSPHVLRNRAQSGSVPQFKKVVFQEFTDGSFTQPLYRGELNEHLGLLGPYIRAEVEDNIMVTFRNQASRPYSFYSSLISYEEDQRQGAEPRKNFVKPNETKTYFWKVQHHMAPTKDEFDCKAWAYFSDVDLEKDVHSGLIGPLLVCHTNTLNPAHGRQVTVQEFALFFTIFDETKSWYFTENMERNCRAPCNIQMEDPTFKENYRFHAINGYIMDTLPGLVMAQDQRIRWYLLSMGSNENIHSIHFSGHVFTVRKKEEYKMALYNLYPGVFETVEMLPSKAGIWRVECLIGEHLHAGMSTLFLVYSNKCQTPLGMASGHIRDFQITASGQYGQWAPKLARLHYSGSINAWSTKEPFSWIKVDLLAPMIIHGIKTQGARQKFSSLYISQFIIMYSLDGKKWQTYRGNSTGTLMVFFGNVDSSGIKHNIFNPPIIARYIRLHPTHYSIRSTLRMELMGCDLNSCSMPLGMESKAISDAQITASSYFTNMFATWSPSKARLHLQGRSNAWRPQVNNPKEWLQVDFQKTMKVTGVTTQGVKSLLTSMYVKEFLISSSQDGHQWTLFFQNGKVKVFQGNQDSFTPVVNSLDPPLLTRYLRIHPQSWVHQIALRMEVLGCEAQDLY

SEQ ID NO: 25 - DNA, 4371 bp, Homo sapiens
atgcaaatagagctctccacctgcttctttctgtgccttttgcgattctgctttagtgccaccagaagatactacctgggtgcagtggaactgtcatgggactatatgcaaagtgatctcggtgagctgcctgtggacgcaagatttcctcctagagtgccaaaatcttttccattcaacacctcagtcgtgtacaaaaagactctgtttgtagaattcacggttcaccttttcaacatcgctaagccaaggccaccctggatgggtctgctaggtcctaccatccaggctgaggtttatgatacagtggtcattacacttaagaacatggcttcccatcctgtcagtcttcatgctgttggtgtatcctactggaaagcttctgagggagctgaatatgatgatcagaccagtcaaagggagaaagaagatgataaagtcttccctggtggaagccatacatatgtctggcaggtcctgaaagagaatggtccaatggcctctgacccactgtgccttacctactcatatctttctcatgtggacctggtaaaagacttgaattcaggcctcattggagccctactagtatgtagagaagggagtctggccaaggaaaagacacagaccttgcacaaatttatactactttttgctgtatttgatgaagggaaaagttggcactcagaaacaaagaactccttgatgcaggatagggatgctgcatctgctcgggcctggcctaaaatgcacacagtcaatggttatgtaaacaggtctctgccaggtctgattggatgccacaggaaatcagtctattggcatgtgattggaatgggcaccactcctgaagtgcactcaatattcctcgaaggtcacacatttcttgtgaggaaccatcgccaggcgtccttggaaatctcgccaataactttccttactgctcaaacactcttgatggaccttggacagtttctactgttttgtcatatctcttcccaccaacatgatggcatggaagcttatgtcaaagtagacagctgtccagaggaaccccaactacgaatgaaaaataatgaagaagcggaagactatgatgatgatcttactgattctgaaatggatgtggtcaggtttgatgatgacaactctccttcctttatccaaattcgctcagttgccaagaagcatcctaaaacttgggtacattacattgctgctgaagaggaggactgggactatgctcccttagtcctcgcccccgatgacagaagttataaaagtcaatatttgaacaatggccctcagcggattggtaggaagtacaaaaaagtccgatttatggcatacacagatgaaacctttaagacgcgtgaagctattcagcatgaatcaggaatcttgggacctttactttatggggaagttggagacacactgttgattatatttaagaatcaagcaagcagaccatataacatctaccctcacggaatcactgatgtccgtcctttgtattcaaggagattaccaaaaggtgtaaaacatttgaaggattttccaattctgccaggagaaatattcaaatataaatggacagtgactgtagaagatgggccaactaaatcagatccgcggtgcctgacccgctattactctagtttcgttaatatggagagagatctagcttcaggactcattggccctctcctcatctgctacaaagaatctgtagatcaaagaggaaaccagataatgtcagacaagaggaatgtcatcctgttttctgtatttgatgagaaccgaagctggtacctcacagagaatatacaacgctttctccccaatccagctggagtgcagcttgaggatccagagttccaagcctccaacatcatgcacagcatcaatggctatgtttttgatagtttgcagttgtcagtttgtttgcatgaggtggcatactggtacattctaagcattggagcacagactgacttcctttctgtcttcttctctggatataccttcaaacacaaaatggtctatgaagacacactcaccctattcccattctcaggagaaactgtcttcatgtcgatggaaaacccaggtctatggattctggggtgccacaactcagactttcggaacagaggcatgaccgccttactgaaggtttctagttgtgacaagaacactggtgattattacgaggacagttatgaagatatttcagcatacttgctgagtaaaaacaatgccattgaacctaggagcttctctcagaatccaccagtcttgaaacgccatcaacgggaaataactcgtactactcttcagtcagatcaagaggaaattgactatgatgataccatatcagttgaaatgaagaaggaagattttgacatttatgatgaggatgaaaatcagagcccccgcagctttcaaaagaaaacacgacactattttattgctgcagtggagaggctctgggattatgggatgagtagctccccacatgttctaagaaacagggctcagagtggcagtgtccctcagttcaagaaagttgttttccaggaatttactgatggctcctttactcagcccttataccgtggagaactaaatgaacatttgggactcctggggccatatataagagcagaagttgaagataatatcatggtaactttcagaaatcaggcctctcgtccctattccttctattctagccttatttcttatgaggaagatcagaggcaaggagcagaacctagaaaaaactttgtcaagcctaatgaaaccaaaacttacttttggaaagtgcaacatcatatggcacccactaaagatgagtttgactgcaaagcctgggcttatttctctgatgttgacctggaaaaagatgtgcactcaggcctgattggaccccttctggtctgccacactaacacactgaaccctgctcatgggagacaagtgacagtacaggaatttgctctgtttttcaccatctttgatgagaccaaaagctggtacttcactgaaaatatggaaagaaactgcagggctccctgcaatatccagatggaagatcccacttttaaagagaattatcgcttccatgcaatcaatggctacataatggatacactacctggcttagtaatggctcaggatcaaaggattcgatggtatctgctcagcatgggcagcaatgaaaacatccattctattcatttcagtggacatgtgttcactgtacgaaaaaaagaggagtataaaatggcactgtacaatctctatccaggtgtttttgagacagtggaaatgttaccatccaaagctggaatttggcgggtggaatgccttattggcgagcatctacatgctgggatgagcacactttttctggtgtacagcaataagtgtcagactcccctgggaatggcttctggacacattagagattttcagattacagcttcaggacaatatggacagtgggccccaaagctggccagacttcattattccggatcaatcaatgcctggagcaccaaggagcccttttcttggatcaaggtggatctgttggcaccaatgattattcacggcatcaagacccagggtgcccgtcagaagttctccagcctctacatctctcagtttatcatcatgtatagtcttgatgggaagaagtggcagacttatcgaggaaattccactggaaccttaatggtcttctttggcaatgtggattcatctgggataaaacacaatatttttaaccctccaattattgctcgatacatccgtttgcacccaactcattatagcattcgcagcactcttcgcatggagttgatgggctgtgatttaaatagttgcagcatgccattgggaatggagagtaaagcaatatcagatgcacagattactgcttcatcctactttaccaatatgtttgccacctggtctccttcaaaagctcgacttcacctccaagggaggagtaatgcctggagacctcaggtgaataatccaaaagagtggctgcaagtggacttccagaagacaatgaaagtcacaggagtaactactcagggagtaaaatctctgcttaccagcatgtatgtgaaggagttcctcatctccagcagtcaagatggccatcagtggactctcttttttcagaatggcaaagtaaaggtttttcagggaaatcaagactccttcacacctgtggtgaactctctagacccaccgttactgactcgctaccttcgaattcacccccagagttgggtgcaccagattgccctgaggatggaggttctgggctgcgaggcacaggacctctac

SEQ ID NO: 26 - protein, 1467 aa, Artificial Sequence
  synthetic HP63/OL aa
MQLELSTCVFLCLLPLGFSAIRRYYLGAVELSWDYRQSELLRELHVDTRFPATAPGALPLGPSVLYKKTVFVEFTDQLFSVARPRPPWMGLLGPTIQAEVYDTVVVTLKNMASHPVSLHAVGVSFWKSSEGAEYEDHTSQREKEDDKVLPGKSQTYVWQVLKENGPTASDPPCLTYSYLSHVDLVKDLNSGLIGALLVCREGSLTRERTQNLHEFVLLFAVFDEGKSWHSARNDSWTRAMDPAPARAQPAMHTVNGYVNRSLPGLIGCHKKSVYWHVIGMGTSPEVHSIFLEGHTFLVRHHRQASLEISPLTFLTAQTFLMDLGQFLLFCHISSHHHGGMEAHVRVESCAEEPQLRRKADEEEDYDDNLYDSDMDVVRLDGDDVSPFIQIRSVAKKHPKTWVHYIAAEEEDWDYAPLVLAPDDRSYKSQYLNNGPQRIGRKYKKVRFMAYTDETFKTREAIQHESGILGPLLYGEVGDTLLIIFKNQASRPYNIYPHGITDVRPLYSRRLPKGVKHLKDFPILPGEIFKYKWTVTVEDGPTKSDPRCLTRYYSSFVNMERDLASGLIGPLLICYKESVDQRGNQIMSDKRNVILFSVFDENRSWYLTENIQRFLPNPAGVQLEDPEFQASNIMHSINGYVFDSLQLSVCLHEVAYWYILSIGAQTDFLSVFFSGYTFKHKMVYEDTLTLFPFSGETVFMSMENPGLWILGCHNSDFRNRGMTALLKVSSCDKNTGDYYEDSYEDISAYLLSKNNAIEPRSFSQNSRHPSTRSQNPPVLKRHQREITRTTLQSDQEEIDYDDTISVEMKKEDFDIYDEDENQSPRSFQKRTRHYFIAAVEQLWDYGMSESPRALRNRAQNGEVPRFKKVVFREFADGSFTQPSYRGELNKHLGLLGPYIRAEVEDNIMVTFKNQASRPYSFYSSLISYPDDQEQGAEPRKNFVKPNETKTYFWKVQHHMAPTEDEFDCKAWAYFSDVDLEKDVHSGLIGPLLICRANTLNAAHGRQVTVQEFALFFTIFDETKSWYFTENVERNCRAPCHLQMEDPTLKENYRFHAINGYVMDTLPGLVMAQNQRIRWYLLSMGSNENIHSIHFSGHVFSVRKKEEYKMAVYNLYPGVFETVEMLPSKVGIWRNRCLIGEHLQAGMSTTFLVYSKKCQTPLGMASGHIRDFQITASGQYGQWAPKLARLHYSGSINAWSTKEPFSWIKVDLLAPMIIHGIKTQGARQKFSSLYISQFIIMYSLDGKKWQTYRGNSTGTLMVFFGNVDSSGIKHNIFNPPIIARYIRLHPTHYSIRSTLRMELMGCDLNSCSMPLGMESKAISDAQITASSYFTNMFATWSPSKARLHLQGRSNAWRPQVNNPKEWLQVDFQKTMKVTGVTTQGVKSLLTSMYVKEFLISSSQDGHQWTLFFQNGKVKVFQGNQDSFTPVVNSLDPPLLTRYLRIHPQSWVHQIALRMEVLGCEAQDLY

SEQ ID NO: 27 - DNA, 4398 bp, Artificial Sequence
  synthetic HP63/OL NT
atgcagctagagctctccacctgtgtctttctgtgtctcttgccactcggctttagtgccatcaggagatactacctgggcgcagtggaactgtcctgggactaccggcaaagtgaactcctccgtgagctgcacgtggacaccagatttcctgctacagcgccaggagctcttccgttgggcccgtcagtcctgtacaaaaagactgtgttcgtagagttcacggatcaacttttcagcgttgccaggcccaggccaccatggatgggtctgctgggtcctaccatccaggctgaggtttacgacacggtggtcgttaccctgaagaacatggcttctcatcccgttagtcttcacgctgtcggcgtctccttctggaaatcttccgaaggcgctgaatatgaggatcacaccagccaaagggagaaggaagacgataaagtccttcccggtaaaagccaaacctacgtctggcaggtcctgaaagaaaatggtccaacagcctctgacccaccatgtcttacctactcatacctgtctcacgtggacctggtgaaagacctgaattcgggcctcattggagccctgctggtttgtagagaagggagtctgaccagagaaaggacccagaacctgcacgaatttgtactactttttgctgtctttgatgaagggaaaagttggcactcagcaagaaatgactcctggacacgggccatggatcccgcacctgccagggcccagcctgcaatgcacacagtcaatggctatgtcaacaggtctctgccaggtctgatcggatgtcataagaaatcagtctactggcacgtgattggaatgggcaccagcccggaagtgcactccatttttcttgaaggccacacgtttctcgtgaggcaccatcgccaggcttccttggagatctcgccactaactttcctcactgctcagacattcctgatggaccttggccagttcctactgttttgtcatatctcttcccaccaccatggtggcatggaggctcacgtcagagtagaaagctgcgccgaggagccccagctgcggaggaaagctgatgaagaggaagattatgatgacaatttgtacgactcggacatggacgtggtccggctcgatggtgacgacgtgtctccctttatccaaatccgctcagttgccaagaagcatcctaaaacttgggtacattacattgctgctgaagaggaggactgggactatgctcccttagtcctcgcccccgatgacagaagttataaaagtcaatatttgaacaatggccctcagcggattggtaggaagtacaaaaaagtccgatttatggcatacacagatgaaacctttaagactcgtgaagctattcagcatgaatcaggaatcttgggacctttactttatggggaagttggagacacactgttgattatatttaagaatcaagcaagcagaccatataacatctaccctcacggaatcactgatgtccgtcctttgtattcaaggagattaccaaaaggtgtaaaacatttgaaggattttccaattctgccaggagaaatattcaaatataaatggacagtgactgtagaagatgggccaactaaatcagatcctcggtgcctgacccgctattactctagtttcgttaatatggagagagatctagcttcaggactcattggccctctcctcatctgctacaaagaatctgtagatcaaagaggaaaccagataatgtcagacaagaggaatgtcatcctgttttctgtatttgatgagaaccgaagctggtacctcacagagaatatacaacgctttctccccaatccagctggagtgcagcttgaggatccagagttccaagcctccaacatcatgcacagcatcaatggctatgtttttgatagtttgcagttgtcagtttgtttgcatgaggtggcatactggtacattctaagcattggagcacagactgacttcctttctgtcttcttctctggatataccttcaaacacaaaatggtctatgaagacacactcaccctattcccattctcaggagaaactgtcttcatgtcgatggaaaacccaggtctatggattctggggtgccacaactcagactttcggaacagaggcatgaccgccttactgaaggtttctagttgtgacaagaacactggtgattattacgaggacagttatgaagatatttcagcatacttgctgagtaaaaacaatgccattgaacctaggagcttctcccagaattcaagacaccctagcactaggtctcaaaacccaccagtcttgaaacgccatcaacgggaaataactcgtactactcttcagtcagatcaagaggaaattgactatgatgataccatatcagttgaaatgaagaaggaagattttgacatttatgatgaggatgaaaatcagagcccccgcagctttcaaaagagaacccgacactatttcattgctgcggtggagcagctctgggattacgggatgagcgaatccccccgggcgctaagaaacagggctcagaacggagaggtgcctcggttcaagaaggtggtcttccgggaatttgctgacggctccttcacgcagccgtcgtaccgcggggaactcaacaaacacttggggctcttgggaccctacatcagagcggaagttgaagacaacatcatggtaactttcaaaaaccaggcgtctcgtccctattccttctactcgagccttatttcttatccggatgatcaggagcaaggggcagaacctcgaaaaaactttgtcaagcctaatgaaaccaaaacttacttttggaaagtgcagcatcacatggcacccacagaagacgagtttgactgcaaagcctgggcctacttttctgatgttgacctggaaaaagatgtgcactcaggcttgatcggcccccttctgatctgccgcgccaacaccctgaacgctgctcacggtagacaagtgaccgtgcaagaatttgctctgtttttcactatttttgatgagacaaagagctggtacttcactgaaaatgtggaaaggaactgccgggccccctgccatctgcagatggaggaccccactctgaaagaaaactatcgcttccatgcaatcaatggctatgtgatggatacactccctggcttagtaatggctcagaatcaaaggatccgatggtatctgctcagcatgggcagcaatgaaaatatccattcgattcattttagcggacacgtgttcagtgtacggaaaaaggaggagtataaaatggccgtgtacaatctctatccgggtgtctttgagacagtggaaatgctaccgtccaaagttggaatttggcggaatagatgcctgattggcgagcacctgcaagctgggatgagcacgactttcctggtgtacagcaagaagtgtcagactcccctgggaatggcttctggacacattagagattttcagattacagcttcaggacaatatggacagtgggccccaaagctggccagacttcattattccggatcaatcaatgcctggagcaccaaggagcccttttcttggatcaaggtggatctgttggcaccaatgattattcacggcatcaagacccagggtgcccgtcagaagttctccagcctctacatctctcagtttatcatcatgtatagtcttgatgggaagaagtggcagacttatcgaggaaattccactggaaccttaatggtcttctttggcaatgtggattcatctgggataaaacacaatatttttaaccctccaattattgctcgatacatccgtttgcacccaactcattatagcattcgcagcactcttcgcatggagttgatgggctgtgatttaaatagttgcagcatgccattgggaatggagagtaaagcaatatcagatgcacagattactgcttcatcctactttaccaatatgtttgccacctggtctccttcaaaagctcgacttcacctccaagggaggagtaatgcctggagacctcaggtgaataatccaaaagagtggctgcaagtggacttccagaagacaatgaaagtcacaggagtaactactcagggagtaaaatctctgcttaccagcatgtatgtgaaggagttcctcatctccagcagtcaagatggccatcagtggactttttttcagaatggcaaagtaaaggtttttcagggaaatcaagactccttcacacctgtggtgaactctctagacccaccgttactgactcgctaccttcgaattcacccccagagttgggtgcaccagattgccctgaggatggaggttctgggctgcgaggcacaggacctctac

SEQ ID NO: 28 - DNA, 5508 bp, Homo sapiens
atgattcctgccagatttgccggggtgctgcttgctctggccctcattttgccagggaccctttgtgcagaaggaactcgcggcaggtcatccacggcccgatgcagccttttcggaagtgacttcgtcaacacctttgatgggagcatgtacagctttgcgggatactgcagttacctcctggcagggggctgccagaaacgctccttctcgattattggggacttccagaatggcaagagagtgagcctctccgtgtatcttggggaattttttgacatccatttgtttgtcaatggtaccgtgacacagggggaccaaagagtctccatgccctatgcctccaaagggctgtatctagaaactgaggctgggtactacaagctgtccggtgaggcctatggctttgtggccaggatcgatggcagcggcaactttcaagtcctgctgtcagacagatacttcaacaagacctgcgggctgtgtggcaactttaacatctttgctgaagatgactttatgacccaagaagggaccttgacctcggacccttatgactttgccaactcatgggctctgagcagtggagaacagtggtgtgaacgggcatctcctcccagcagctcatgcaacatctcctctggggaaatgcagaagggcctgtgggagcagtgccagcttctgaagagcacctcggtgtttgcccgctgccaccctctggtggaccccgagccttttgtggccctgtgtgagaagactttgtgtgagtgtgctggggggctggagtgcgcctgccctgccctcctggagtacgcccggacctgtgcccaggagggaatggtgctgtacggctggaccgaccacagcgcgtgcagcccagtgtgccctgctggtatggagtataggcagtgtgtgtccccttgcgccaggacctgccagagcctgcacatcaatgaaatgtgtcaggagcgatgcgtggatggctgcagctgccctgagggacagctcctggatgaaggcctctgcgtggagagcaccgagtgtccctgcgtgcattccggaaagcgctaccctcccggcacctccctctctcgagactgcaacacctgcatttgccgaaacagccagtggatctgcagcaatgaagaatgtccaggggagtgccttgtcacaggtcaatcacacttcaagagctttgacaacagatacttcaccttcagtgggatctgccagtacctgctggcccgggattgccaggaccactccttctccattgtcattgagactgtccagtgtgctgatgaccgcgacgctgtgtgcacccgctccgtcaccgtccggctgcctggcctgcacaacagccttgtgaaactgaagcatggggcaggagttgccatggatggccaggacgtccagctccccctcctgaaaggtgacctccgcatccagcatacagtgacggcctccgtgcgcctcagctacggggaggacctgcagatggactgggatggccgcgggaggctgctggtgaagctgtcccccgtctatgccgggaagacctgcggcctgtgtgggaattacaatggcaaccagggcgacgacttccttaccccctctgggctggcggagccccgggtggaggacttcgggaacgcctggaagctgcacggggactgccaggacctgcagaagcagcacagcgatccctgcgccctcaacccgcgcatgaccaggttctccgaggaggcgtgcgcggtcctgacgtcccccacattcgaggcctgccatcgtgccgtcagcccgctgccctacctgcggaactgccgctacgacgtgtgctcctgctcggacggccgcgagtgcctgtgcggcgccctggccagctatgccgcggcctgcgcggggagaggcgtgcgcgtcgcgtggcgcgagccaggccgctgtgagctgaactgcccgaaaggccaggtgtacctgcagtgcgggaccccctgcaacctgacctgccgctctctctcttacccggatgaggaatgcaatgaggcctgcctggagggctgcttctgccccccagggctctacatggatgagaggggggactgcgtgcccaaggcccagtgcccctgttactatgacggtgagatcttccagccagaagacatcttctcagaccatcacaccatgtgctactgtgaggatggcttcatgcactgtaccatgagtggagtccccggaagcttgctgcctgacgctgtcctcagcagtcccctgtctcatcgcagcaaaaggagcctatcctgtcggccccccatggtcaagctggtgtgtcccgctgacaacctgcgggctgaagggctcgagtgtaccaaaacgtgccagaactatgacctggagtgcatgagcatgggctgtgtctctggctgcctctgccccccgggcatggtccggcatgagaacagatgtgtggccctggaaaggtgtccctgcttccatcagggcaaggagtatgcccctggagaaacagtgaagattggctgcaacacttgtgtctgtcgggaccggaagtggaactgcacagaccatgtgtgtgatgccacgtgctccacgatcggcatggcccactacctcaccttcgacgggctcaaatacctgttccccggggagtgccagtacgttctggtgcaggattactgcggcagtaaccctgggacctttcggatcctagtggggaataagggatgcagccacccctcagtgaaatgcaagaaacgggtcaccatcctggtggagggaggagagattgagctgtttgacggggaggtgaatgtgaagaggcccatgaaggatgagactcactttgaggtggtggagtctggccggtacatcattctgctgctgggcaaagccctctccgtggtctgggaccgccacctgagcatctccgtggtcctgaagcagacataccaggagaaagtgtgtggcctgtgtgggaattttgatggcatccagaacaatgacctcaccagcagcaacctccaagtggaggaagaccctgtggactttgggaactcctggaaagtgagctcgcagtgtgctgacaccagaaaagtgcctctggactcatcccctgccacctgccataacaacatcatgaagcagacgatggtggattcctcctgtagaatccttaccagtgacgtcttccaggactgcaacaagctggtggaccccgagccatatctggatgtctgcatttacgacacctgctcctgtgagtccattggggactgcgcctgcttctgcgacaccattgctgcctatgcccacgtgtgtgcccagcatggcaaggtggtgacctggaggacggccacattgtgcccccagagctgcgaggagaggaatctccgggagaacgggtatgagtgtgagtggcgctataacagctgtgcacctgcctgtcaagtcacgtgtcagcaccctgagccactggcctgccctgtgcagtgtgtggagggctgccatgcccactgccctccagggaaaatcctggatgagcttttgcagacctgcgttgaccctgaagactgtccagtgtgtgaggtggctggccggcgttttgcctcaggaaagaaagtcaccttgaatcccagtgaccctgagcactgccagatttgccactgtgatgttgtcaacctcacctgtgaagcctgccaggagccgggaggcctggtggtgcctcccacagatgccccggtgagccccaccactctgtatgtggaggacatctcggaaccgccgttgcacgatttctactgcagcaggctactggacctggtcttcctgctggatggctcctccaggctgtccgaggctgagtttgaagtgctgaaggcctttgtggtggacatgatggagcggctgcgcatctcccagaagtgggtccgcgtggccgtggtggagtaccacgacggctcccacgcctacatcgggctcaaggaccggaagcgaccgtcagagctgcggcgcattgccagccaggtgaagtatgcgggcagccaggtggcctccaccagcgaggtcttgaaatacacactgttccaaatcttcagcaagatcgaccgccctgaagcctcccgcatcaccctgctcctgatggccagccaggagccccaacggatgtcccggaactttgtccgctacgtccagggcctgaagaagaagaaggtcattgtgatcccggtgggcattgggccccatgccaacctcaagcagatccgcctcatcgagaagcaggcccctgagaacaaggccttcgtgctgagcagtgtggatgagctggagcagcaaagggacgagatcgttagctacctctgtgaccttgcccctgaagcccctcctcctactctgccccccgacatggcacaagtcactgtgggcccggggctcttgggggtttcgaccctggggcccaagaggaactccatggttctggatgtggcgttcgtcctggaaggatcggacaaaattggtgaagccgacttcaacaggagcaaggagttcatggaggaggtgattcagcggatggatgtgggccaggacagcatccacgtcacggtgctgcagtactcctacatggtgactgtggagtaccccttcagcgaggcacagtccaaaggggacatcctgcagcgggtgcgagagatccgctaccagggcggcaacaggaccaacactgggctggccctgcggtacctctctgaccacagcttcttggtcagccagggtgaccgggagcaggcgcccaacctggtctacatggtcaccggaaatcctgcctctgatgagatcaagaggctgcctggagacatccaggtggtgcccattggagtgggccctaatgccaacgtgcaggagctggagaggattggctggcccaatgcccctatcctcatccaggactttgagacgctcccccgagaggctcctgacctggtgctgcagaggtgctgctccggagaggggctgcagatccccaccctctcccctgcacctcgtgatgagacgctccaggatggctgtgatactcacttctgcaaggtcaatgagagaggagagtacttctgggagaagagggtcacaggctgcccaccctttgatgaacacaagtgtctggctgagggaggtaaaattatgaaaattccaggcacctgctgtgacacatgtgaggagcctgagtgcaacgacatcactgccaggctgcagtatgtcaaggtgggaagctgtaagtctgaagtagaggtggatatccactactgccagggcaaatgtgccagcaaagccatgtactccattgacatcaacgatgtgcaggaccagtgctcctgctgctctccgacacggacggagcccatgcaggtggccctgcactgcaccaatggctctgttgtgtaccatgaggttctcaatgccatggagtgcaaatgctcccccaggaagtgcagcaagtga

SEQ ID NO: 29 - DNA, 6648 bp, Ovis aries
atgtttcccaccaggctcgcgaggctgctgcttgctgtggccctcactttgccaggggccctttgtggagaaggtgctcctggcaagtcatcgatggcccggtgcagcctcttcggagctgacttcatcaacacctttgatgagagcatgtacagctttgcgggagactgtagttacctcctggcaggggattgcaagacacactccttttcaatcgtaggggacttccaagctggtagaagagtgggtctctctgtgtaccttggggaatttttcgacatccatgtgtttgtcaacggtactgtgctgcaggggggccagcatgtctccatgccctatgccaccagagggctgtacctggacaccgaggctgggtaccacaagctgtccagcgagtcttatggctttgtggccaggatcgacagcagcgggaacttccaaatcctgctgtcggacagacacttcaacaagacctgtgggctgtgcggtgactttaacatcttcgccgaagatgacttcaggactcaagaaggaaccctgacctcagacccctacgactttgcaaactcctgggccctgagcagtgaggagcagcggtgtccacgggtgtcccctcccagcagctcctgcaacatctcctctgagctgcagaagggcctgtgggagcagtgccagcttctgaagacggcctccgtgttcgcccgctgccacgccctggtggaccccgagcctttcgtggccctgtgtgagcggatgctgtgcgcatgcgcccaggggctgcgctgcccctgcccggtgctcctggagtacgcccgcgcctgcgcccagcaagggatgctgctgtacggctgggcggaccacagctcctgccgaccggactgccccgcgggcatggagtacaaggagtgtgtgtccccatgccacaggacctgccggagcctgagtatcaccgaagtgtgtcgggagcagtgtgtggatggctgcagctgccctgagggacagctcctggatgaaggccgctgtgtggaaagtgccgagtgtccctgtgtgcatgctggaaagccataccctcctggcgcctccctctcgcgagactgcaacacctgcatctgccgaaacagccagtgggtctgcagcaatgaggactgtccaggagagtgtctcatcacaggacaatcccacttcaagagctttgacgacaggcacttcaccttcagcggggtctgccagtacctgctggcccaggactgccaggaccactccttctccgtcatcatagagactgttcagtgtgctgacgaccctgatgcggtctgcacccgctccgtcaccgtccgcctgcccagcccgcaccacggcctcctgaagctgaagcacgggggtggagtcgccctggatggccaggacgtccagattcccctcctgcaaggtgacctccggatccagcacactgtgacggcctccctgcacctcatcttcggggaggacctgcagatagactgggacggtcgcgggaggctgctgctgaagctgtccccggtctacgcggggaggacctgcgggctgtgcgggaattacaacggcaaccagagggatgacttcctgacgcccgcgggcctggtcgagcccctggtggagcactttggaaactcctggaagctacgtgcagactgtgaggacttgcaggagcagcccagtgacccctgcagcctcaacccgcgcctgaccaagttcgcagaccaggcctgcgccatcctgacgtcccgcaagttcgaggcctgccacagcgccgtgggcccgctgccctacctgcgcaactgccgcttcgacgtgtgcgcctgctccgatggcagagactgcctgtgcgacgcggtggccaactacgcggcggcctgcgccaggaggggcgtgcacatcgggtggcgggagcccagcttctgtgcactgagctgcccacacggccaggtgtaccagcagtgtgggaccccctgcaacctcacctgccgctcactctcccacccggacgaggaatgcactgaggtctgtctggagggctgcttctgccctgctgggctcttcctggatgagacggggtcctgtgtgcccaaggcccagtgcccctgttactatgacggcgagatcttccaacctgaagacatcttctcggaccatcacaccatgtgctactgcgaagatggcttcatgcactgctccacgagcggagccccggggagcctgctgcctgaagcagtcctcagcagccctctgtcccaccgcagcaaaaggagcctgtcctgccggccccccatggtcaagctggtgtgccctgctgacaacccgagggccgaagggctcgaatgcaccaagacctgccagaactatgacctggaatgcgtgagcacgggctgtgtgtccggctgcctctgccccccgggcatggtccggcatgagaacaggtgtgtggccctggaaaggtgcccctgcttccaccagggcagagagtacgcccccggagacagggtgaaggccgactgcaacacctgcgtctgtcaggaccggaagtggaactgtacggaccgcgtgtgtgatgctggctgctctgccgtgggcctggctcactacttcacctttgatgggctcaagtacctgttcccgggggagtgccagtacgtcctggtacaggaccactgcggtagtaaccctgggaccttccgggtcctggtggggaatgaggggtgcagcgtcccctccctgaagtgcaggaagcgcatcaccatcctggtggagggaggagagatcgagctgtttgacggggaggtgaacgtgaagaagcccatgaaggatgagacgcacttcgaggtggtggaatctggccggtacatcactgtgctgctgggcaaggccctctctgtggtctgggacgggcacctggccatctctgtgttcctgaagcggatgtaccaggagcgggtatgcggcctgtgtgggaatttcgatggcgtccagaacaatgacctcaccagtagcagcctccaagtggaggaagaccctgtggactttgggaattcctggaaagtgagcccgcattgcgctgacacccagaaagtgccgctggactcggcccctgccacctgccacaagaacgtcatgaagcagaccatggtggattcctcctgcagggtcctcaccagtgatgttttccgggagtgcaacaggctggtgaaccccgagccgtacctggatgtttgcatctacgacagctgctcctgcgagtccatcggggactgcgcctgcttctgtgacaccatcgccgcctacgcccacgagtgtgcccagcacggcgaagtggtgacctggaggacagccacactgtgcccccagaattgtgaggagcggaacctgaaggagagtgggtaccaatgtgagtggcgctacaacagctgtgctcccgcctgtccagtcacgtgccagcacccagagcccctggcctgccccgtgcagtgcgtggagggctgccacgcacactgcccgcctgggaaaatcctggacgagcttttgcagacctgtgtcaaccccgaggactgccctgtgtgccaggtggagggccggcgcttagcctccgggaagaaagtgaccctgaaccctggggaccctgagcattgccagctctgtcactgtgatggtgtcagcctcacttgtgaagcctgcagggagccaggaggcctgcccgtgccccccaccgaaggcccggtcagccccacaaccccgtacgtggaggacaccccggagccacccctgcacgacttcttctgcagcaaactgctggacctggtcttcctgctggacggctcctccaagctgtctgaggccgacttcgagacgctgaaggcgttcgtggtgggcatgatggagcgtctgcacatttcccagaaacgcatccgtgtggccgtggtggagtaccacgatggctcccatgcctaccttgcactgcaagaccggaagcggccatccgagctgcggcgcattgccgggcaggtgaagtacgcgggcagcgaggtggcttccaccagcgaggtcttgaagtacacgctcttccagatcttcggcaggattgaccggcccgaggcctctcgcgtggccctgctgcttacggccagccaggagccccccaggctggcccggaacttggtccgctacctccagggcctgaagaagaagaaggtctccgtggtcccggtgggcatcgggccccacgtcagcctcaagcagatccgcctcatcgagaagcaggcgtctgagaacaaagcctttgtgctaagcggtgtgcacgagctggagcagcggatgaacgagattgtcggctacctctgtgacctcgcccccgaggtgcctgccccgaccccgacgcgacatcctctcattgcgcaggtcactgtggcgccgcagctcctgggtccttcgccaccaggacccaagaggagctctgtggtcctggatgtggcattcctcctggaaggctcggatgaggtaggcgaggccaacttcaacaggagcgcagagtttgtggaggaggtgatccgacgcatggacgttggccgggacggcatccatgtcacggtgctgcagtactcgtacacggtgaccgtggagcactcgttcagggagccacagtccaaggaggtggtcctgcagcgactccatgaagtccgctaccggggtggcaaccagacgaacacggggctggccctgcagtacctgtcggagcacagcttctccgccagccagggggaccgggagcaggcgcccaacctggtctacatggtgacgggcagcccggcctcggacaagatccagcggatgccaggagacatccagctcgtgcccatcggcgtgggcccccgtgtggacgtgcaggagctggagagggtcagctggccccagacccccatcttcatccaggacttcgagaggctcccccgagaagctccggatctggtgctgcagcggtgctgctccgaagacggcccgcacctccccaccctcgcccctgccccagactgcagccagcccctggatgtagtcctcctcctggatggctcctccacccctccagcctcttactttgacgaaatgaagagtttcgccaaggctttcatctcaaaagccaacctaggccctcagcttacccaggtgtcagtcctgcagtacgggagcatcaccaacgtcgacgtatcctggaatgtgcacgtggacaaagcccacctgctgagccttgtggaccccatgcagcgcgagggaggccccagccgagtcggggaggcgttgtccttcgcggtgcgctacatcacgtcccaagtccacggtgccaggcccggggcctccaaggtggtggtgatcctggtcacaggctcctccatggactcagtggaggcggccgccgctgctgccagatccaaccgagtggctgtgttccccatcgggatcggggaccagtatgacgcagcccagctgagggtcttggcgggcccgggggccagctccaatgtggcagagctccagcggattgaagacctccccagcatggttgcccttggcaactccttcttccagaggctatgctctgggttcgtcagtgtttgcgtggatgaggacgggaatgagaggaggcctggggacgtctggaccttgctggatcagtgccacacagtgacttgcctgccagatggccagaccttgctgaagagtcaccgggtcaactgtgatcaggggccacagccatcatgccccgacggccagatcccgctcaggatggaggaagcctgtggctgccgctgggcctgtccctgtgtgtgcacaggcagctccactcggcacatcgtgacctttgatggacggaatttcaagctgaccggcaactgctcatacgttctgtttcacaacaaggagcaggacttggaggtgattctccataacggattctgcagcgctggggcgaggcaggcctgcatgaaatctgtggaggtgaagcacagcggcctctcggttgagctccgcagcaacatggaggtgatggtgaatgggagactggtctctgtcccttacctgggtggggacatggaggtcagagtctatggtaccatcatgttcgaggtcagattcaaccttctgggccacatcctctccttcaccccacgtgatgagacactccaggatggctgtgacagtcacttctgcaaagtcaacaagagaggagagttcatttgggagaagagggtcatgggctgcccgcccttcaacgaacacaaatgtctggctgagggggggaaagtcatgaaaattcctggcacgtgctgtgacacatgtgaggagcccgagtgcaaggacatcacagccagggtgcagtacatcaaggtgggagactgcaaatctgaagaggaagtggacattaactactgccagggaagatgcaccagcaaagccctgtactccatcgacacggaggacgtgcaagaccagtgttcctgctgctcgcccacgcgcacggagcccatgtcagtgcccctgcgctgcaccaacggctccatcattcaccatgtgatcctcaacgccctgcagtgcaagtgctcatccaggaagtgccgcccgtga

SEQ ID NO: 30 - protein, 24 aa, Artificial Sequence
  synthetic porcine-derived linker sequence
SFAQNSRPPSASAPKPPVLRRHQR

SEQ ID NO: 31 - protein, 14 aa, Artificial Sequence
  synthetic human linker sequence
SFSQNPPVLKRHQR

SEQ ID NO: 32 - protein, 6 aa, Artificial Sequence
  synthetic 6-His tag
HHHHHH

SEQ ID NO: 33 - DNA, 4350 bp, Artificial Sequence
  Synthetic truncated ovine (sheep) gene
atgcacatcaagctctgtacctgcctctttctgtgcctctggccatgcagcttcagtgccatcagaagatactacctgggtgcagtggaactgtcctgggactatacgcgaagtgaactgctcagtgagctgcatgtgaacacgaggtttcctcccagagtgcccaaaccttttccattcaacacatcagtcatgtacagaaagactgtgtttgtagagttcacggatcaactttttaacatcgccaagcccaggccaccatggatgggtctgctgggtccagctatccaggctgaggtttatgacaccgtggtcattacatttaagaatatggcttctcatcctgttagtcttcatgctattggcgtatcctactggaaatcttctgaaggtgctgcatataaggatgaaaccagccaaagggagaaggaagatgacaaagtcattcctggtaaaagtcatacctacgtctggcatatcctgaaagaaaacggtccaacagcctctgacccaccatgtctcacctactcatatctttctcatgtggacctggtgaaagacgtgaactcaggtctcatcggagccctgctaatttgtagggaagggactctgatcaaagaaaggacacagaccttgcacaaattcgtactactgtttgctgtatttgatgaagggaaaagttggcactcgggaaaaaatgagtccttgacacatgttatggattctgcctctgtactgcacaccatcaatggctatataaacaggtctctgccaggtctgattggatgtcataagaaatcagtctattggcatgtgattggaatgggcaccaccccagaagtgcactcaattttcctcgaaggccacacatttctcgtgaggaaccatcgccaggcttccttggagatctcaccaataactttccttaccgctcagacagtcctgatggactgtggccagtttctactgttttgtcgtatctcttcccaccaacatgatggtatggaagcttatgtcaaagtagatagttgcccagaggaaccccgactatggatgaaaaataaccaagaagaagattacgatgatggtttggatgactctgacatggatgtggtcaggttcgatggtgacagtgtgcctccctttatccaaatgcgctcagttgcaaagaagcatcctaaaacctgggtccactacattgctgctgaagaggatgactgggactatgccccctcggtcctcacctccaatgacagaagttataaaagtctgtatctgaaccacggtcctcagcggattggtaggaagtacagaaaagtacgatttatagcttacacagatggaacatttaagactcgtgaagctattcagcatgaatcagggatcctggggcctttactttatggagaagttggagacacacttttgattatatttaagaatcaagcaagccggccatataacatctaccctcatggaatcactgatgtcagtcctttgcactcagggagatttccaaaaggtgtgaaacatttgaaagacatgccaattctgccaggagaagtgttcaagtataaatggacagtgactgtagaagatgggccaactaaatcagatcctcggtgtctgacccgatattactcgagtttcattaacttagagaaagatctagcttcaggactcattggccccctcctcatctgttacaaagaatctgtagatcaaagaggaaaccagatgatgtcagacaagagaaatgtcatcctgttttctgtatttgatgaaaacaaaagttggtacctcacagagaatattcaacgcttcctccccagtggagtacagccccaggatccagagttccaagtctccaatgtcatgcacagcatcaatggctatgtttttgatagcttgcagctgtcggtttgtttgcatgaggtggcgtactggtacattctaagtgttggagcccaaattgacttcctctctgtcttcttctctggatataccttcaaacacaaaatggtctatgaagacacactcaccctattccccttctcgggagaaactgtcttcatgtcaatggaaaatccaggtctgtgggttctggggtgccacaactcagactttcgaaacagaggcatgacagccttactgaaggttgatagttgtgacaggaacgttggcgattattatgacacatatgaagctattccaaccttcctgctgagtgaaaacaatgtcattgaacccagaagcttctcccagaatccaccaagcttgaaacgccatcaaagggagataacccttactacttttcagccagagccagacaaaactgactatgatgatactttgtcgattgaaacaaagagagaagattttgacatttatggtgaagatgaaaatcaggacccccgcagctttcaaaagagaacacgccactattttattgctgcagtggagcggctctgggattatgggatgagtagatccccccacgcactaagaaacaggtctcagaatggaggagtccctcagttcaaaaaggtggtgttcgaggaatttactgatggctcctttactcaggccgtataccgtggacaattaaatgaacacctgggactcttgggaccatatataagagcagaagtggaagacaatatcatggtaactttcaaaaaccaggcctctcgtccctactccttctattctagccttatttcttataacggagatcagagacaaggagcagaacctcgaaaaaagtttgtcaagcctaatgaaacccaaagctacttttggaaagtgcagcaccatatggcacccaccaaagatgagtttgactgcaaagcctgggcttacttttctgatgttgatctggaaaaagatgtgcactcaggcttgattggccccattctgatctgccgtgtggacacgctgagtgctgctcatgggagacaagtgacagtacaggaattcgctctgtttttcaccatttttgatgagaccaagagctggtactttgccgaaaacatggcaaggaactgcgtggcaccctgccatgtccagccagaggaccctactttccaagaaaagtatcgcttccatgcaatcaatggctacgtgatggatacactccctggcttagtcatggctcagcatcaaaggattaggtggtatctgctcagcatgggcagcaatgaaaatatccattccattcatttcagtggccatgtgttcactgtgagaaaaacggaggagtataaaatggcggtctacaatctctacccaggtgtctttgagaccgtggaaatgctaccatccaaggttgggacttggcggatagaatgtcttattggcgagcacctacaagctgggatgagcactctcttcctggtgtacagcaaggagtgtcaaattccactgggaatggcttctggacgcattagagattttcagattacagcttcaggacaatatggacagtgggccccaaagctggccagacttcattattctggatcaatcaatgcctggagcaccaaggatccctctccttggatcaaggtggatctgttggcgccgatgattattcacagcatcctgactcagggtgcccggcagaagttctccagcctgtacatctctcagtttatcatcatgtacagcctcgatggacagcggtggcagggttatcgggggaactccactgggactttaatggtgttctttggcaatgtggattcatctggagtaaaacacaatatttttaaccctccaattattgctagatatatccgtttgcacccaacgcattacagcatccgcagcactcttcgcatggagttgatgggctgtgacttaaatagttgcaacatgccactgggaatggagaataaagctatatcagatacacagattactgcctcatcccacttaagcaacatgtttgccacctggtctccttcacaagcccgacttaaccttcaagggaggacaaatgcctggagaccccaggtgaataatccaaaagagtggctacaagtggacttccagaagacaatgagagttacaggaataaccactcaaggggtgaaatctctgcttaccagcatgtatgtgaaggagttccttatatccagtagtcaagagggccataactggactccatttcttcagaatggcaaagtgaaggtttttcagggaaatcaagactccttcacccccgtggtgaatactctagaccccccactgtttacccgcttccttcggattcacccgcagagctgggtgcaccatatcgccctgaggctggagttttggggttgtgaggcacagcagcagtactag